European Patent Specification EP 3 511 339 B1, published April 9, 2025. Title: Polypeptides. Applicant: Swedish Orphan Biovitrum AB. The sequence listing filed with the application follows.

SEQUENCE LISTING (762 sequences)

SEQ ID NO: 1 - protein, 29 aa, artificial sequence
  Modified bacterial sequence
EVLEAWDEIDRLPNLTIEQWLAFINKLDD

SEQ ID NO: 2 - protein, 29 aa, artificial sequence
  Modified bacterial sequence
EVLEAWNEIDRLPNLTIEQWLAFINKLDD

SEQ ID NO: 3 - protein, 29 aa, artificial sequence
  Modified bacterial sequence
EVIEAWNEIDRLPNLTIEQWLAFINKLDD

SEQ ID NO: 4 - protein, 29 aa, artificial sequence
  Modified bacterial sequence
EVLEAWDEIDRLPNLTLDQWLAFINKLDD

SEQ ID NO: 5 - protein, 29 aa, artificial sequence
  Modified bacterial sequence
EVLDAWDEIDALPNLTLEQWLAFINKLDD

SEQ ID NO: 6 - protein, 29 aa, artificial sequence
  Modified bacterial sequence
EVIDAWDEIDRLPNLTLDQWLAFINKLDD

SEQ ID NO: 7 - protein, 29 aa, artificial sequence
  Modified bacterial sequence
ETLEAWDEIDRLPNLTIEQWLAFINKLDD

SEQ ID NO: 8 - protein, 29 aa, artificial sequence
  Modified bacterial sequence
EVIDAWNEIDALPNLTLDQWLAFINKLDD

SEQ ID NO: 9 - protein, 29 aa, artificial sequence
  Modified bacterial sequence
EVLDAWDEIDKLPNLTIDQWLAFINKLDD

SEQ ID NO: 10 - protein, 29 aa, artificial sequence
  Modified bacterial sequence
EVLEAWDEIDHLPNLTLDQWLAFINKLDD

SEQ ID NO: 11 - protein, 29 aa, artificial sequence
  Modified bacterial sequence
EVLEAWDEIDALPNLTIEQWLAFINKLDD

SEQ ID NO: 12 - protein, 29 aa, artificial sequence
  Modified bacterial sequence
EVLDAWDEIDKLPNLTLEQWLAFINKLDD

SEQ ID NO: 13 - protein, 29 aa, artificial sequence
  Modified bacterial sequence
ETITAWDEIDKLPNLTIEQWLAFIGKLED

SEQ ID NO: 14 - protein, 29 aa, artificial sequence
  Modified bacterial sequence
ESMKAWDEIDRLPNLNINQWVAFIDSLYD

SEQ ID NO: 15 - protein, 29 aa, artificial sequence
  Modified bacterial sequence
ESIEAWTEIDHLPNLTIEQWLAFINKLTD

SEQ ID NO: 16 - protein, 29 aa, artificial sequence
  Modified bacterial sequence
EVLDAWHEIDTLPNLTVRQWLAFISKLED

SEQ ID NO: 17 - protein, 29 aa, artificial sequence
  Modified bacterial sequence
EHIQANEEIDRLPNLTIKQWLAFINKLHD

SEQ ID NO: 18 - protein, 29 aa, artificial sequence
  Modified bacterial sequence
EVLHAWAEIDALPNLTIEQWLAFINKLDD

SEQ ID NO: 19 - protein, 29 aa, artificial sequence
  Modified bacterial sequence
EVLAAWDEIDSLPNLTLQQWLAFINKLDD

SEQ ID NO: 20 - protein, 29 aa, artificial sequence
  Modified bacterial sequence
EVIDAWNEIDALPNLTLEQWLAFINKLDD

SEQ ID NO: 21 - protein, 29 aa, artificial sequence
  Modified bacterial sequence
EVLDAWNEIDALPNLTIDQWLAFINKLSD

SEQ ID NO: 22 - protein, 29 aa, artificial sequence
  Modified bacterial sequence
EVIEAWDEIDGLPNLTIEQWLAFINKLDD

SEQ ID NO: 23 - protein, 29 aa, artificial sequence
  Modified bacterial sequence
EVLEAWDEIDHLPNLTLQQWLAFINKLDD

SEQ ID NO: 24 - protein, 29 aa, artificial sequence
  Modified bacterial sequence
EVIEAWNEIDALPNLTIEQWLAFINKLDD

SEQ ID NO: 25 - protein, 29 aa, artificial sequence
  Modified bacterial sequence
EVIAAWNEIDRLPNLTLTQWLAFINKLDD

SEQ ID NO: 26 - protein, 29 aa, artificial sequence
  Modified bacterial sequence
EVIEAWDEIDALPNLTLQQWLAFINKLDD

SEQ ID NO: 27 - protein, 29 aa, artificial sequence
  Modified bacterial sequence
EVIAAWDEIDKLPNLTIEQWLAFINKLDD

SEQ ID NO: 28 - protein, 29 aa, artificial sequence
  Modified bacterial sequence
EVIAAWDEIDKLPNLTLQQWLAFINKLDD

SEQ ID NO: 29 - protein, 29 aa, artificial sequence
  Modified bacterial sequence
ETIAAWDEIDKLPNLTIEQWLAFINKLDD

SEQ ID NO: 30 - protein, 29 aa, artificial sequence
  Modified bacterial sequence
ETIEAWNEIDRLPNLTIEQWLAFINKLDD

SEQ ID NO: 31 - protein, 29 aa, artificial sequence
  Modified bacterial sequence
EVLEAWREIDALPNLTIQQWLAFINKLDD

SEQ ID NO: 32 - protein, 29 aa, artificial sequence
  Modified bacterial sequence
EVIEAWDEIDQLPNLTIEQWLAFINKLDD

SEQ ID NO: 33 - protein, 29 aa, artificial sequence
  Modified bacterial sequence
EVLRAWDEIDHLPNLTLEQWLAFINKLDD

SEQ ID NO: 34 - protein, 29 aa, artificial sequence
  Modified bacterial sequence
EVLEAWDEIDRLPNLTLNQWLAFINKLDD

SEQ ID NO: 35 - protein, 29 aa, artificial sequence
  Modified bacterial sequence
EVLDAWNEIDHLPNLTIEQWLAFINKLDD

SEQ ID NO: 36 - protein, 29 aa, artificial sequence
  Modified bacterial sequence
EVIDAWNEIDKLPNLTIEQWLAFINKLDD

SEQ ID NO: 37 - protein, 29 aa, artificial sequence
  Modified bacterial sequence
ETLEAWDEIDQLPNLTLQQWLAFINKLDD

SEQ ID NO: 38 - protein, 29 aa, artificial sequence
  Modified bacterial sequence
EVIEAWNEIDALPNLTLDQWLAFINKLDD

SEQ ID NO: 39 - protein, 29 aa, artificial sequence
  Modified bacterial sequence
EVIDAWNEIDRLPNLTLQQWLAFINKLDD

SEQ ID NO: 40 - protein, 29 aa, artificial sequence
  Modified bacterial sequence
EVIDAWNEIDQLPNLTLEQWLAFINKLDD

SEQ ID NO: 41 - protein, 29 aa, artificial sequence
  Modified bacterial sequence
ETIAAWDEIDHLPNLTLEQWLAFINKLDD

SEQ ID NO: 42 - protein, 29 aa, artificial sequence
  Modified bacterial sequence
EVLQAWDEIDHLPNLTIQQWLAFINKLSD

SEQ ID NO: 43 - protein, 29 aa, artificial sequence
  Modified bacterial sequence
ETLHAWAEIDRLPNLTIEQWLAFINKLDD

SEQ ID NO: 44 - protein, 29 aa, artificial sequence
  Modified bacterial sequence
EVLEAWNEIDHLPNLTLAQWLAFINKLDD

SEQ ID NO: 45 - protein, 29 aa, artificial sequence
  Modified bacterial sequence
EVIEAWDEIDKLPNLTIAQWLAFINKLDD

SEQ ID NO: 46 - protein, 29 aa, artificial sequence
  Modified bacterial sequence
EVLDAWDEIDHLPNLTLQQWLAFINKLDD

SEQ ID NO: 47 - protein, 29 aa, artificial sequence
  Modified bacterial sequence
ETIEAWNEIDKLPNLTLTQWLAFINKLDD

SEQ ID NO: 48 - protein, 29 aa, artificial sequence
  Modified bacterial sequence
EVLEAWNEIDLLPNLTIEQWLAFINKLDD

SEQ ID NO: 49 - protein, 29 aa, artificial sequence
  Modified bacterial sequence
EVIEAWDEIDHLPNLTIDQWLAFINKLDD

SEQ ID NO: 50 - protein, 29 aa, artificial sequence
  Modified bacterial sequence
EVISAWNEIDALPNLTLQQWLAFINKLDD

SEQ ID NO: 51 - protein, 29 aa, artificial sequence
  Modified bacterial sequence
EVIAAWNEIDKLPNLTLEQWLAFINKLDD

SEQ ID NO: 52 - protein, 29 aa, artificial sequence
  Modified bacterial sequence
ETIEAWNEIDSLPNLTLDQWLAFINKLDD

SEQ ID NO: 53 - protein, 29 aa, artificial sequence
  Modified bacterial sequence
EVLDAWNEIDQLPNLTLQQWLAFINKLDD

SEQ ID NO: 54 - protein, 29 aa, artificial sequence
  Modified bacterial sequence
EVLAAWNEIDHLPNLTIEQWLAFINKLDD

SEQ ID NO: 55 - protein, 29 aa, artificial sequence
  Modified bacterial sequence
EVLEAWDEIDHLPNLTITQWLAFINKLDD

SEQ ID NO: 56 - protein, 29 aa, artificial sequence
  Modified bacterial sequence
ETIDAWNEIDHLPNLTIEQWLAFINKLDD

SEQ ID NO: 57 - protein, 29 aa, artificial sequence
  Modified bacterial sequence
EVIEAWNEIDHLPNLTIQQWLAFINKLDD

SEQ ID NO: 58 - protein, 29 aa, artificial sequence
  Modified bacterial sequence
EVIQAWNEIDALPNLTISQWLAFINKLDD

SEQ ID NO: 59 - protein, 29 aa, artificial sequence
  Modified bacterial sequence
EVIAAWDEIDSLPNLTIEQWLAFINKLDD

SEQ ID NO: 60 - protein, 29 aa, artificial sequence
  Modified bacterial sequence
EHIEAWNEIDALPNLTIEQWLAFINKLQD

SEQ ID NO: 61 - protein, 29 aa, artificial sequence
  Modified bacterial sequence
EVLEAWNEIDKLPNLTLDQWLAFINKLDD

SEQ ID NO: 62 - protein, 29 aa, artificial sequence
  Modified bacterial sequence
EVIDAWNEIDHLPNLTIEQWLAFINKLAD

SEQ ID NO: 63 - protein, 29 aa, artificial sequence
  Modified bacterial sequence
ETIDAWDEIDKLPNLTIEQWLAFINKLDD

SEQ ID NO: 64 - protein, 29 aa, artificial sequence
  Modified bacterial sequence
EVIAAWDEIDLLPNLTLQQWLAFINKLAD

SEQ ID NO: 65 - protein, 29 aa, artificial sequence
  Modified bacterial sequence
EVIHAWDEIDKLPNLTIEQWLAFINKLDD

SEQ ID NO: 66 - protein, 29 aa, artificial sequence
  Modified bacterial sequence
EVIAAWNEIDHLPNLTLEQWLAFINKLDD

SEQ ID NO: 67 - protein, 29 aa, artificial sequence
  Modified bacterial sequence
ETLDAWNEIDKLPNLTLSQWLAFINKLDD

SEQ ID NO: 68 - protein, 29 aa, artificial sequence
  Modified bacterial sequence
EVLEAWNEIDALPNLTLEQWLAFINKLDD

SEQ ID NO: 69 - protein, 29 aa, artificial sequence
  Modified bacterial sequence
EVIQAWDEIDHLPNLTISQWLAFINKLDD

SEQ ID NO: 70 - protein, 29 aa, artificial sequence
  Modified bacterial sequence
EVLQAWDEIDSLPNLTIEQWLAFINKLDD

SEQ ID NO: 71 - protein, 29 aa, artificial sequence
  Modified bacterial sequence
ETLEAWDEIDHLPNLTIAQWLAFINKLDD

SEQ ID NO: 72 - protein, 29 aa, artificial sequence
  Modified bacterial sequence
ETIDAWNEIDRLPNLTISQWLAFINKLDD

SEQ ID NO: 73 - protein, 29 aa, artificial sequence
  Modified bacterial sequence
EVLDAWHEIDHLPNLTIQQWLAFINKLDD

SEQ ID NO: 74 - protein, 29 aa, artificial sequence
  Modified bacterial sequence
EQIRAWDEIDKLPNLTIEQWLAFINKLAD

SEQ ID NO: 75 - protein, 29 aa, artificial sequence
  Modified bacterial sequence
ETLYAWNEIDKLPNLTIEQWLAFIEKLQD

SEQ ID NO: 76 - protein, 29 aa, artificial sequence
  Modified bacterial sequence
EVIEAWNEIDALPNLTIDQWLAFINKLDD

SEQ ID NO: 77 - protein, 29 aa, artificial sequence
  Modified bacterial sequence
EVLEAWNEIDHLPNLTIQQWLAFINKLDD

SEQ ID NO: 78 - protein, 29 aa, artificial sequence
  Modified bacterial sequence
ETIEAWDEIDALPNLTIEQWLAFINKLDD

SEQ ID NO: 79 - protein, 29 aa, artificial sequence
  Modified bacterial sequence
EVIEAWNEIDHLPNLTLQQWLAFINKLDD

SEQ ID NO: 80 - protein, 29 aa, artificial sequence
  Modified bacterial sequence
EVIEAWNEIDKLPNLTIQQWLAFINKLDD

SEQ ID NO: 81 - protein, 29 aa, artificial sequence
  Modified bacterial sequence
ETLDAWAEIDHLPNLTLDQWLAFINKLDD

SEQ ID NO: 82 - protein, 29 aa, artificial sequence
  Modified bacterial sequence
EHIDAWNEIDALPNLTLSQWLAFINKLDD

SEQ ID NO: 83 - protein, 29 aa, artificial sequence
  Modified bacterial sequence
EVLDAWNEIDKLPNLTIAQWLAFINKLDD

SEQ ID NO: 84 - protein, 29 aa, artificial sequence
  Modified bacterial sequence
EVIEAWTEIDYLPNLTLQQWLAFINKLDD

SEQ ID NO: 85 - protein, 29 aa, artificial sequence
  Modified bacterial sequence
ETIEAWNEIDHLPNLTIAQWLAFINKLDD

SEQ ID NO: 86 - protein, 29 aa, artificial sequence
  Modified bacterial sequence
EVIQAWNEIDKLPNLTLEQWLAFINKLDD

SEQ ID NO: 87 - protein, 29 aa, artificial sequence
  Modified bacterial sequence
EVIEAWDEIDHLPNLTIEQWLAFINKLDD

SEQ ID NO: 88 - protein, 29 aa, artificial sequence
  Modified bacterial sequence
ETIDAWNEIDLLPNLTIEQWLAFINKLDD

SEQ ID NO: 89 - protein, 29 aa, artificial sequence
  Modified bacterial sequence
EHIDAWNEIDKLPNLTLDQWLAFINKLDD

SEQ ID NO: 90 - protein, 29 aa, artificial sequence
  Modified bacterial sequence
EVVAAWNEIDALPNLTIEQWLAFINKLND

SEQ ID NO: 91 - protein, 29 aa, artificial sequence
  Modified bacterial sequence
EVIEAWNEIDALPNLTLAQWLAFINKLDD

SEQ ID NO: 92 - protein, 29 aa, artificial sequence
  Modified bacterial sequence
EVLQAWDEIDRLPNLTLDQWLAFINKLDD

SEQ ID NO: 93 - protein, 29 aa, artificial sequence
  Modified bacterial sequence
EVIDAWDEIDHLPNLTIEQWLAFINKLSD

SEQ ID NO: 94 - protein, 29 aa, artificial sequence
  Modified bacterial sequence
EVVEAWNEIDQLPNLTIEQWLAFINKLDD

SEQ ID NO: 95 - protein, 29 aa, artificial sequence
  Modified bacterial sequence
EVIQAWNEIDALPNLTIEQWLAFINKLDD

SEQ ID NO: 96 - protein, 29 aa, artificial sequence
  Modified bacterial sequence
EVIQAWDEIDKLPNLTIDQWLAFINKLAD

SEQ ID NO: 97 - protein, 29 aa, artificial sequence
  Modified bacterial sequence
EVVAAWDEIDALPNLTLTQWLAFINKLDD

SEQ ID NO: 98 - protein, 29 aa, artificial sequence
  Modified bacterial sequence
EVIQAWNEIDGLPNLTLSQWLAFINKLDD

SEQ ID NO: 99 - protein, 29 aa, artificial sequence
  Modified bacterial sequence
ETIEAWDEIDALPNLTITQWLAFINKLDD

SEQ ID NO: 100 - protein, 29 aa, artificial sequence
  Modified bacterial sequence
EVIDAWNEIDHLPNLTIQQWLAFINKLAD

SEQ ID NO: 101 - protein, 29 aa, artificial sequence
  Modified bacterial sequence
ETIEAWNEIDALPNLTLDQWLAFINKLED

SEQ ID NO: 102 - protein, 29 aa, artificial sequence
  Modified bacterial sequence
EHIHAWNEIDELPNLTIEQWLAFINKLAD

SEQ ID NO: 103 - protein, 29 aa, artificial sequence
  Modified bacterial sequence
EVIDAWDEIDHLPNLTIDQWLAFINKLSD

SEQ ID NO: 104 - protein, 29 aa, artificial sequence
  Modified bacterial sequence
EVIDANDEIDALPNLTIAQWLAFINKLHD

SEQ ID NO: 105 - protein, 29 aa, artificial sequence
  Modified bacterial sequence
ETIEAWDEIDKLPNLTIEQWLAFINKLDD

SEQ ID NO: 106 - protein, 29 aa, artificial sequence
  Modified bacterial sequence
EVLLAWDEIDHLPNLTLEQWLAFINKLDD

SEQ ID NO: 107 - protein, 29 aa, artificial sequence
  Modified bacterial sequence
EHIDAWNEIDGLPNLTLEQWLAFINKLDD

SEQ ID NO: 108 - protein, 29 aa, artificial sequence
  Modified bacterial sequence
EVIEAWSEIDALPNLTIDQWLAFINKLAD

SEQ ID NO: 109 - protein, 29 aa, artificial sequence
  Modified bacterial sequence
EQLNAWAEIDALPNLTIEQWLAFINKLDD

SEQ ID NO: 110 - protein, 29 aa, artificial sequence
  Modified bacterial sequence
EVIDAWNEIDALPNLTIAQWLAFINKLDD

SEQ ID NO: 111 - protein, 29 aa, artificial sequence
  Modified bacterial sequence
ETIDAWNEIDQLPNLTIEQWLAFINKLDD

SEQ ID NO: 112 - protein, 29 aa, artificial sequence
  Modified bacterial sequence
EVIEAWDEIDKLPNLTLAQWLAFINKLDD

SEQ ID NO: 113 - protein, 29 aa, artificial sequence
  Modified bacterial sequence
EVLYAWAEIDHLPNLTIEQWLAFINKLDD

SEQ ID NO: 114 - protein, 29 aa, artificial sequence
  Modified bacterial sequence
EQIDAWNEIDRLPNLTIQQWLAFINKLDD

SEQ ID NO: 115 - protein, 29 aa, artificial sequence
  Modified bacterial sequence
EVLAAWDEIDRLPNLTIEQWLAFINKLDD

SEQ ID NO: 116 - protein, 29 aa, artificial sequence
  Modified bacterial sequence
EVIEAWDEIDHLPNLTLHQWLAFINKLDD

SEQ ID NO: 117 - protein, 29 aa, artificial sequence
  Modified bacterial sequence
EVIEAWNEIDKLPNLTLQQWLAFINKLDD

SEQ ID NO: 118 - protein, 29 aa, artificial sequence
  Modified bacterial sequence
EVIDANDEIDALPNLTIEQWLAFINKLHD

SEQ ID NO: 119 - protein, 29 aa, artificial sequence
  Modified bacterial sequence
EVIAAWDEIDALPNLTIEQWLAFINKLDD

SEQ ID NO: 120 - protein, 29 aa, artificial sequence
  Modified bacterial sequence
EVIEAWTEIDQLPNLTLDQWLAFINKLDD

SEQ ID NO: 121 - protein, 29 aa, artificial sequence
  Modified bacterial sequence
EVINAWNEIDALPNLTLQQWLAFINKLDD

SEQ ID NO: 122 - protein, 29 aa, artificial sequence
  Modified bacterial sequence
EHIEAWDEIDHLPNLTIDQWLAFINKLAD

SEQ ID NO: 123 - protein, 29 aa, artificial sequence
  Modified bacterial sequence
EHLEAWREIDALPNLTIEQWLAFINKLDD

SEQ ID NO: 124 - protein, 29 aa, artificial sequence
  Modified bacterial sequence
EVLDAWNEIDKLPNLTLQQWLAFINKLDD

SEQ ID NO: 125 - protein, 29 aa, artificial sequence
  Modified bacterial sequence
EVIAAWDEIDHLPNLTIQQWLAFINKLDD

SEQ ID NO: 126 - protein, 29 aa, artificial sequence
  Modified bacterial sequence
EVIQAWNEIDALPNLTLEQWLAFINKLDD

SEQ ID NO: 127 - protein, 29 aa, artificial sequence
  Modified bacterial sequence
EVIDAWNEIDHLPNLTIAQWLAFINKLDD

SEQ ID NO: 128 - protein, 29 aa, artificial sequence
  Modified bacterial sequence
EQLDAWDEIDHLPNLTIDQWLAFINKLSD

SEQ ID NO: 129 - protein, 29 aa, artificial sequence
  Modified bacterial sequence
EVLNAWDEIDKLPNLTIEQWLAFINKLDD

SEQ ID NO: 130 - protein, 29 aa, artificial sequence
  Modified bacterial sequence
EVLEAWNEIDHLPNLTIDQWLAFINKLDD

SEQ ID NO: 131 - protein, 29 aa, artificial sequence
  Modified bacterial sequence
EVLLAWDEIDRLPNLTIDQWLAFINKLAD

SEQ ID NO: 132 - protein, 29 aa, artificial sequence
  Modified bacterial sequence
EVIAAWNEIDQLPNLTLDQWLAFINKLDD

SEQ ID NO: 133 - protein, 29 aa, artificial sequence
  Modified bacterial sequence
ETLLAWDEIDALPNLTIEQWLAFINKLDD

SEQ ID NO: 134 - protein, 29 aa, artificial sequence
  Modified bacterial sequence
EVIDAWNEIDTLPNLTLEQWLAFINKLDD

SEQ ID NO: 135 - protein, 29 aa, artificial sequence
  Modified bacterial sequence
EVLHAWNEIDHLPNLTLNQWLAFINKLQD

SEQ ID NO: 136 - protein, 29 aa, artificial sequence
  Modified bacterial sequence
EVIQAWNEIDALPNLTIAQWLAFINKLDD

SEQ ID NO: 137 - protein, 29 aa, artificial sequence
  Modified bacterial sequence
ETVDAWNEIDALPNLTIEQWLAFINKLDD

SEQ ID NO: 138 - protein, 29 aa, artificial sequence
  Modified bacterial sequence
EVIQAWDEIDHLPNLTIDQWLAFINKLDD

SEQ ID NO: 139 - protein, 29 aa, artificial sequence
  Modified bacterial sequence
EVLDAWNEIDQLPNLTIQQWLAFINKLDD

SEQ ID NO: 140 - protein, 29 aa, artificial sequence
  Modified bacterial sequence
ETIEAWNEIDALPNLTLDQWLAFINKLDD

SEQ ID NO: 141 - protein, 29 aa, artificial sequence
  Modified bacterial sequence
EVIEAWDEIDALPNLTIDQWLAFINKLDD

SEQ ID NO: 142 - protein, 29 aa, artificial sequence
  Modified bacterial sequence
EVIEAWNEIDQLPNLTIQQWLAFINKLDD

SEQ ID NO: 143 - protein, 29 aa, artificial sequence
  Modified bacterial sequence
EVIEAWTEIDHLPNLTIEQWLAFINKLDD

SEQ ID NO: 144 - protein, 29 aa, artificial sequence
  Modified bacterial sequence
EVIQAWNEIDHLPNLTLQQWLAFINKLED

SEQ ID NO: 145 - protein, 29 aa, artificial sequence
  Modified bacterial sequence
EVIQANNEIDQLPNLTIEQWLAFINKLHD

SEQ ID NO: 146 - protein, 29 aa, artificial sequence
  Modified bacterial sequence
EVLHAWSEIDKLPNLTIEQWLAFINKLDD

SEQ ID NO: 147 - protein, 29 aa, artificial sequence
  Modified bacterial sequence
ETIQAWDEIDKLPNLTLDQWLAFINKLSD

SEQ ID NO: 148 - protein, 29 aa, artificial sequence
  Modified bacterial sequence
ETLRAWDEIDKLPNLTIQQWLAFINKLAD

SEQ ID NO: 149 - protein, 29 aa, artificial sequence
  Modified bacterial sequence
EVIDAWNEIDHLPNLTIEQWLAFINKLED

SEQ ID NO: 150 - protein, 29 aa, artificial sequence
  Modified bacterial sequence
EVIDAWNEIDHLPNLTLQQWLAFINKLAD

SEQ ID NO: 151 - protein, 29 aa, artificial sequence
  Modified bacterial sequence
ETIDAWNEIDALPNLTLDQWLAFINKLDD

SEQ ID NO: 152 - protein, 29 aa, artificial sequence
  Modified bacterial sequence
EVIEAWNEIDQLPNLTIEQWLAFINKLDD

SEQ ID NO: 153 - protein, 29 aa, artificial sequence
  Modified bacterial sequence
EVIRAWDEIDQLPNLTLSQWLAFINKLDD

SEQ ID NO: 154 - protein, 29 aa, artificial sequence
  Modified bacterial sequence
EVIEAWNEIDRLPNLTIHQWLAFINKLDD

SEQ ID NO: 155 - protein, 29 aa, artificial sequence
  Modified bacterial sequence
ETIEAWNEIDQLPNLTIEQWLAFINKLDD

SEQ ID NO: 156 - protein, 29 aa, artificial sequence
  Modified bacterial sequence
EVLTAWAEIDALPNLTLSQWLAFINKLDD

SEQ ID NO: 157 - protein, 29 aa, artificial sequence
  Modified bacterial sequence
EVIEAWDEIDKLPNLTVDQWLAFINKLDD

SEQ ID NO: 158 - protein, 29 aa, artificial sequence
  Modified bacterial sequence
EVIDAWNEIDHLPNLTLTQWLAFINKLDD

SEQ ID NO: 159 - protein, 29 aa, artificial sequence
  Modified bacterial sequence
EVIEAWNEIDQLPNLTLDQWLAFINKLDD

SEQ ID NO: 160 - protein, 29 aa, artificial sequence
  Modified bacterial sequence
ETLQAWDEIDHLPNLTLNQWLAFINKLDD

SEQ ID NO: 161 - protein, 29 aa, artificial sequence
  Modified bacterial sequence
EVIDAWNEIDHLPNLTIEQWLAFINKLDD

SEQ ID NO: 162 - protein, 29 aa, artificial sequence
  Modified bacterial sequence
EVIEAWNEIDLLPNLTLSQWLAFINKLDD

SEQ ID NO: 163 - protein, 29 aa, artificial sequence
  Modified bacterial sequence
EVIDAWDEIDRLPNLTLKQWLAFINKLDD

SEQ ID NO: 164 - protein, 29 aa, artificial sequence
  Modified bacterial sequence
ETLHAWDEIDKLPNLTIEQWLAFINKLDD

SEQ ID NO: 165 - protein, 29 aa, artificial sequence
  Modified bacterial sequence
EVIKAWDEIDHLPNLTLNQWLAFINKLDD

SEQ ID NO: 166 - protein, 29 aa, artificial sequence
  Modified bacterial sequence
EVIEAWNEIDHLPNLTLAQWLAFINKLDD

SEQ ID NO: 167 - protein, 29 aa, artificial sequence
  Modified bacterial sequence
EVIQAWNEIDHLPNLTIDQWLAFITKLED

SEQ ID NO: 168 - protein, 29 aa, artificial sequence
  Modified bacterial sequence
EVIEAWNEIDRLPNLTIKQWLAFINKLDD

SEQ ID NO: 169 - protein, 29 aa, artificial sequence
  Modified bacterial sequence
EVIEAWNEIDSLPNLTLQQWLAFINKLDD

SEQ ID NO: 170 - protein, 29 aa, artificial sequence
  Modified bacterial sequence
ETIDAWNEIDKLPNLTIEQWLAFINKLDD

SEQ ID NO: 171 - protein, 29 aa, artificial sequence
  Modified bacterial sequence
EVLEAWAEIDALPNLTIAQWLAFINKLDD

SEQ ID NO: 172 - protein, 29 aa, artificial sequence
  Modified bacterial sequence
ETIDAWNEIDRLPNLTIEQWLAFINKLDD

SEQ ID NO: 173 - protein, 29 aa, artificial sequence
  Modified bacterial sequence
ETLKAWDEIDRLPNLTLEQWLAFINKLDD

SEQ ID NO: 174 - protein, 29 aa, artificial sequence
  Modified bacterial sequence
ETIAAWNEIDALPNLTLQQWLAFINKLDD

SEQ ID NO: 175 - protein, 29 aa, artificial sequence
  Modified bacterial sequence
EVLQAWNEIDHLPNLTIQQWLAFINKLDD

SEQ ID NO: 176 - protein, 29 aa, artificial sequence
  Modified bacterial sequence
EVIEAWSEIDHLPNLTLQQWLAFINKLDD

SEQ ID NO: 177 - protein, 29 aa, artificial sequence
  Modified bacterial sequence
EVIDAWNEIDGLPNLTIEQWLAFINKLDD

SEQ ID NO: 178 - protein, 29 aa, artificial sequence
  Modified bacterial sequence
EVIHAWNEIDHLPNLTLNQWLAFINKLED

SEQ ID NO: 179 - protein, 29 aa, artificial sequence
  Modified bacterial sequence
EVLDAWNEIDSLPNLTLDQWLAFINKLDD

SEQ ID NO: 180 - protein, 29 aa, artificial sequence
  Modified bacterial sequence
EQIEAWNEIDRLPNLTLEQWLAFINKLDD

SEQ ID NO: 181 - protein, 29 aa, artificial sequence
  Modified bacterial sequence
EVVDAWNEIDALPNLTLQQWLAFINKLDD

SEQ ID NO: 182 - protein, 29 aa, artificial sequence
  Modified bacterial sequence
EVIEAWNEIDKLPNLTIEQWLAFINKLDD

SEQ ID NO: 183 - protein, 29 aa, artificial sequence
  Modified bacterial sequence
EVIEANDEIDRLPNLTIEQWLAFINKLHD

SEQ ID NO: 184 - protein, 29 aa, artificial sequence
  Modified bacterial sequence
ETLQAWDEIDKLPNLTIEQWLAFINKLDD

SEQ ID NO: 185 - protein, 29 aa, artificial sequence
  Modified bacterial sequence
EVIEAWDEIDHLPNLTIDQWLAFINKLAD

SEQ ID NO: 186 - protein, 29 aa, artificial sequence
  Modified bacterial sequence
ETIDAWNEIDHLPNLTLQQWLAFINKLAD

SEQ ID NO: 187 - protein, 29 aa, artificial sequence
  Modified bacterial sequence
EVIDAWDEIDKLPNLTIEQWLAFINKLDD

SEQ ID NO: 188 - protein, 29 aa, artificial sequence
  Modified bacterial sequence
EVIEAWNEIDKLPNLTLAQWLAFINKLDD

SEQ ID NO: 189 - protein, 29 aa, artificial sequence
  Modified bacterial sequence
EVLQAWDEIDKLPNLTIQQWLAFINKLDD

SEQ ID NO: 190 - protein, 29 aa, artificial sequence
  Modified bacterial sequence
EVIAAWNEIDGLPNLTLQQWLAFINKLDD

SEQ ID NO: 191 - protein, 29 aa, artificial sequence
  Modified bacterial sequence
ETLNAWNEIDALPNLTLQQWLAFINKLDD

SEQ ID NO: 192 - protein, 29 aa, artificial sequence
  Modified bacterial sequence
EVLSAWNEIDQLPNLTLEQWLAFINKLDD

SEQ ID NO: 193 - protein, 29 aa, artificial sequence
  Modified bacterial sequence
ETLEAWDEIDHLPNLTLHQWLAFINKLDD

SEQ ID NO: 194 - protein, 29 aa, artificial sequence
  Modified bacterial sequence
EQIEAWNEIDHLPNLTLQQWLAFINKLAD

SEQ ID NO: 195 - protein, 29 aa, artificial sequence
  Modified bacterial sequence
EVVEAWDEIDKLPNLTIEQWLAFINKLDD

SEQ ID NO: 196 - protein, 29 aa, artificial sequence
  Modified bacterial sequence
EVLEAWNEIDELPNLTIEQWLAFINKLDD

SEQ ID NO: 197 - protein, 29 aa, artificial sequence
  Modified bacterial sequence
EVIDAWNEIDQLPNLTLQQWLAFINKLDD

SEQ ID NO: 198 - protein, 29 aa, artificial sequence
  Modified bacterial sequence
ETIDAWDEIDKLPNLTLSQWLAFINKLDD

SEQ ID NO: 199 - protein, 29 aa, artificial sequence
  Modified bacterial sequence
ETIDAWNEIDQLPNLTLQQWLAFINKLDD

SEQ ID NO: 200 - protein, 29 aa, artificial sequence
  Modified bacterial sequence
EVIQAWDEIDALPNLTLNQWLAFINKLDD

SEQ ID NO: 201 - protein, 29 aa, artificial sequence
  Modified bacterial sequence
EVLDAWAEIDQLPNLTLQQWLAFINKLDD

SEQ ID NO: 202 - protein, 29 aa, artificial sequence
  Modified bacterial sequence
EHIAAWDEIDALPNLTIEQWLAFINKLDD

SEQ ID NO: 203 - protein, 29 aa, artificial sequence
  Modified bacterial sequence
EVIRAWDEIDALPNLTIEQWLAFINKLDD

SEQ ID NO: 204 - protein, 29 aa, artificial sequence
  Modified bacterial sequence
EVIDAWDEIDALPNLTIDQWLAFINKLAD

SEQ ID NO: 205 - protein, 29 aa, artificial sequence
  Modified bacterial sequence
EVIDAWNEIDRLPNLTIQQWLAFINKLDD

SEQ ID NO: 206 - protein, 29 aa, artificial sequence
  Modified bacterial sequence
EVITAWNEIDHLPNLTLSQWLAFINKLDD

SEQ ID NO: 207 - protein, 29 aa, artificial sequence
  Modified bacterial sequence
EVIDAWNEIDALPNLTIHQWLAFINKLDD

SEQ ID NO: 208 - protein, 29 aa, artificial sequence
  Modified bacterial sequence
EQLKAWDEIDKLPNLTIEQWLAFIEKLQD

SEQ ID NO: 209 - protein, 29 aa, artificial sequence
  Modified bacterial sequence
EHIDAWTEIDHLPNLTIEQWLAFINKLDD

SEQ ID NO: 210 - protein, 29 aa, artificial sequence
  Modified bacterial sequence
EQLRAWDEIDKLPNLTIEQWLAFINKLQD

SEQ ID NO: 211 - protein, 29 aa, artificial sequence
  Modified bacterial sequence
EVLEAWREIDSLPNLTIAQWLAFINKLDD

SEQ ID NO: 212 - protein, 29 aa, artificial sequence
  Modified bacterial sequence
EVIQAWNEIDKLPNLTIEQWLAFINKLDD

SEQ ID NO: 213 - protein, 29 aa, artificial sequence
  Modified bacterial sequence
EHVEAWNEIDQLPNLTIEQWLAFINKLAD

SEQ ID NO: 214 - protein, 29 aa, artificial sequence
  Modified bacterial sequence
EVIDAWDEIDALPNLTIDQWLAFINKLSD

SEQ ID NO: 215 - protein, 29 aa, artificial sequence
  Modified bacterial sequence
EVIEAWNEIDHLPNLTIEQWLAFINKLDD

SEQ ID NO: 216 - protein, 29 aa, artificial sequence
  Modified bacterial sequence
EVLQAWDEIDKLPNLTIEQWLAFINKLSD

SEQ ID NO: 217 - protein, 29 aa, artificial sequence
  Modified bacterial sequence
EVIKAWNEIDSLPNLTIEQWLAFINKLDD

SEQ ID NO: 218 - protein, 29 aa, artificial sequence
  Modified bacterial sequence
EVLEAWHEIDLLPNLTIQQWLAFINKLDD

SEQ ID NO: 219 - protein, 29 aa, artificial sequence
  Modified bacterial sequence
EVLEAWTEIDRLPNLTLDQWLAFINKLDD

SEQ ID NO: 220 - protein, 29 aa, artificial sequence
  Modified bacterial sequence
EQLYAWNEIDHLPNLTIEQWLAFIEKLQD

SEQ ID NO: 221 - protein, 29 aa, artificial sequence
  Modified bacterial sequence
EVLNAWDEIDKLPNLTIKQWLAFINKLDD

SEQ ID NO: 222 - protein, 29 aa, artificial sequence
  Modified bacterial sequence
EVIRAWDEIDKLPNLTVEQWLAFINKLDD

SEQ ID NO: 223 - protein, 29 aa, artificial sequence
  Modified bacterial sequence
EVVQAWDEIDQLPNLTLEQWLAFINKLDD

SEQ ID NO: 224 - protein, 29 aa, artificial sequence
  Modified bacterial sequence
EVIRAWDEIDQLPNLTLEQWLAFINKLDD

SEQ ID NO: 225 - protein, 29 aa, artificial sequence
  Modified bacterial sequence
ETIDAWNEIDHLPNLTLDQWLAFINKLDD

SEQ ID NO: 226 - protein, 29 aa, artificial sequence
  Modified bacterial sequence
EVVAAWTEIDLLPNLTLDQWLAFINKLED

SEQ ID NO: 227 - protein, 29 aa, artificial sequence
  Modified bacterial sequence
EVVAAWDEIDALPNLTIEQWLAFINKLSD

SEQ ID NO: 228 - protein, 29 aa, artificial sequence
  Modified bacterial sequence
ETLEAWREIDSLPNLTLEQWLAFINKLDD

SEQ ID NO: 229 - protein, 29 aa, artificial sequence
  Modified bacterial sequence
EVIKAWNEIDHLPNLTLDQWLAFINKLDD

SEQ ID NO: 230 - protein, 29 aa, artificial sequence
  Modified bacterial sequence
EVLEAWTEIDKLPNLTIDQWLAFINKLDD

SEQ ID NO: 231 - protein, 29 aa, artificial sequence
  Modified bacterial sequence
ETLEAWDEIDKLPNLTIDQWLAFINKLDD

SEQ ID NO: 232 - protein, 29 aa, artificial sequence
  Modified bacterial sequence
EVIEAWNEIDKLPNLTIDQWLAFINKLDD

SEQ ID NO: 233 - protein, 29 aa, artificial sequence
  Modified bacterial sequence
ETIDAWNEIDKLPNLTLEQWLAFINKLDD

SEQ ID NO: 234 - protein, 29 aa, artificial sequence
  Modified bacterial sequence
ETLDAWDEIDALPNLTIDQWLAFINKLED

SEQ ID NO: 235 - protein, 29 aa, artificial sequence
  Modified bacterial sequence
EVLSAWNEIDHLPNLTIQQWLAFINKLDD

SEQ ID NO: 236 - protein, 29 aa, artificial sequence
  Modified bacterial sequence
EVIQANDEIDKLPNLTIEQWLAFIHKLHD

SEQ ID NO: 237 - protein, 29 aa, artificial sequence
  Modified bacterial sequence
EHLDAWDEIDHLPNLTIQQWLAFINKLAD

SEQ ID NO: 238 - protein, 29 aa, artificial sequence
  Modified bacterial sequence
EVIQAWNEIDQLPNLTIEQWLAFINKLDD

SEQ ID NO: 239 - protein, 29 aa, artificial sequence
  Modified bacterial sequence
EVIEAWNEIDYLPNLTIAQWIAFINKLDD

SEQ ID NO: 240 - protein, 29 aa, artificial sequence
  Modified bacterial sequence
ETIQAWDEIDRLPNLTLQQWLAFINKLDD

SEQ ID NO: 241 - protein, 29 aa, artificial sequence
  Modified bacterial sequence
ETIQAWDEIDKLPNLTIEQWLAFINKLDD

SEQ ID NO: 242 - protein, 29 aa, artificial sequence
  Modified bacterial sequence
ETLDAWAEIDHLPNLTIEQWLAFINKLDD

SEQ ID NO: 243 - protein, 29 aa, artificial sequence
  Modified bacterial sequence
EVIEAWDEIDKLPNLTLNQWLAFINKLDD

SEQ ID NO: 244 - protein, 29 aa, artificial sequence
  Modified bacterial sequence
EVLDAWNEIDQLPNLTIEQWLAFINKLDD

SEQ ID NO: 245 - protein, 29 aa, artificial sequence
  Modified bacterial sequence
EVLHAWNEIDHLPNLTIEQWLAFIEKLED

SEQ ID NO: 246 - protein, 29 aa, artificial sequence
  Modified bacterial sequence
EVIEAWQEIDKLPNLTIDQWLAFINKLDD

SEQ ID NO: 247 - protein, 29 aa, artificial sequence
  Modified bacterial sequence
EVVDAWNEIDQLPNLTIEQWLAFINKLDD

SEQ ID NO: 248 - protein, 29 aa, artificial sequence
  Modified bacterial sequence
EQIEAWNEIDALPNLTIEQWLAFINKLAD

SEQ ID NO: 249 - protein, 49 aa, artificial sequence
  Modified bacterial sequence
KEVLEAWDEIDRLPNLTIEQWLAFINKLDDDPSQSSELLSEAKKLNDSQ

SEQ ID NO: 250 - protein, 49 aa, artificial sequence
  Modified bacterial sequence
KEVLEAWNEIDRLPNLTIEQWLAFINKLDDDPSQSSELLSEAKKLNDSQ

SEQ ID NO: 251 - protein, 49 aa, artificial sequence
  Modified bacterial sequence
KEVIEAWNEIDRLPNLTIEQWLAFINKLDDDPSQSSELLSEAKKLNDSQ

SEQ ID NO: 252 - protein, 49 aa, artificial sequence
  Modified bacterial sequence
KEVLEAWDEIDRLPNLTLDQWLAFINKLDDDPSQSSELLSEAKKLNDSQ

SEQ ID NO: 253 - protein, 49 aa, artificial sequence
  Modified bacterial sequence
KEVLDAWDEIDALPNLTLEQWLAFINKLDDDPSQSSELLSEAKKLNDSQ

SEQ ID NO: 254 - protein, 49 aa, artificial sequence
  Modified bacterial sequence
KEVIDAWDEIDRLPNLTLDQWLAFINKLDDDPSQSSELLSEAKKLNDSQ

SEQ ID NO: 255 - protein, 49 aa, artificial sequence
  Modified bacterial sequence
KETLEAWDEIDRLPNLTIEQWLAFINKLDDDPSQSSELLSEAKKLNDSQ

SEQ ID NO: 256 - protein, 49 aa, artificial sequence
  Modified bacterial sequence
KEVIDAWNEIDALPNLTLDQWLAFINKLDDDPSQSSELLSEAKKLNDSQ

SEQ ID NO: 257 - protein, 49 aa, artificial sequence
  Modified bacterial sequence
KEVLDAWDEIDKLPNLTIDQWLAFINKLDDDPSQSSELLSEAKKLNDSQ

SEQ ID NO: 258 - protein, 49 aa, artificial sequence
  Modified bacterial sequence
KEVLEAWDEIDHLPNLTLDQWLAFINKLDDDPSQSSELLSEAKKLNDSQ

SEQ ID NO: 259 - protein, 49 aa, artificial sequence
  Modified bacterial sequence
KEVLEAWDEIDALPNLTIEQWLAFINKLDDDPSQSSELLSEAKKLNDSQ

SEQ ID NO: 260 - protein, 49 aa, artificial sequence
  Modified bacterial sequence
KEVLDAWDEIDKLPNLTLEQWLAFINKLDDDPSQSSELLSEAKKLNDSQ

SEQ ID NO: 261 - protein, 49 aa, artificial sequence
  Modified bacterial sequence
KETITAWDEIDKLPNLTIEQWLAFIGKLEDDPSQSSELLAEAKKLNDAQ

SEQ ID NO: 262 - protein, 49 aa, artificial sequence
  Modified bacterial sequence
KESMKAWDEIDRLPNLNINQWVAFIDSLYDDPSQSANLLAEAKKLNDAQ

SEQ ID NO: 263 - protein, 49 aa, artificial sequence
  Modified bacterial sequence
KESIEAWTEIDHLPNLTIEQWLAFINKLTDDPSQSSELLAEAKKLNDAQ

SEQ ID NO: 264 - protein, 49 aa, artificial sequence
  Modified bacterial sequence
KEVLDAWHEIDTLPNLTVRQWLAFISKLEDDPSQSSELLAEAKKLNDAQ

SEQ ID NO: 265 - protein, 49 aa, artificial sequence
  Modified bacterial sequence
KEHIQANEEIDRLPNLTIKQWLAFINKLHDDPSQSSELLAEAKKLNDAQ

SEQ ID NO: 266 - protein, 49 aa, artificial sequence
  Modified bacterial sequence
KEVLHAWAEIDALPNLTIEQWLAFINKLDDDPSQSSELLSEAKKLNDSQ

SEQ ID NO: 267 - protein, 49 aa, artificial sequence
  Modified bacterial sequence
KEVLAAWDEIDSLPNLTLQQWLAFINKLDDDPSQSSELLSEAKKLNDSQ

SEQ ID NO: 268 - protein, 49 aa, artificial sequence
  Modified bacterial sequence
KEVIDAWNEIDALPNLTLEQWLAFINKLDDDPSQSSELLSEAKKLNDSQ

SEQ ID NO: 269 - protein, 49 aa, artificial sequence
  Modified bacterial sequence
KEVLDAWNEIDALPNLTIDQWLAFINKLSDDPSQSSELLSEAKKLNDSQ

SEQ ID NO: 270 - protein, 49 aa, artificial sequence
  Modified bacterial sequence
KEVIEAWDEIDGLPNLTIEQWLAFINKLDDDPSQSSELLSEAKKLNDSQ

SEQ ID NO: 271 - protein, 49 aa, artificial sequence
  Modified bacterial sequence
KEVLEAWDEIDHLPNLTLQQWLAFINKLDDDPSQSSELLSEAKKLNDSQ

SEQ ID NO: 272 - protein, 49 aa, artificial sequence
  Modified bacterial sequence
KEVIEAWNEIDALPNLTIEQWLAFINKLDDDPSQSSELLSEAKKLNDSQ

SEQ ID NO: 273 - protein, 49 aa, artificial sequence
  Modified bacterial sequence
KEVIAAWNEIDRLPNLTLTQWLAFINKLDDDPSQSSELLSEAKKLNDSQ

SEQ ID NO: 274 - protein, 49 aa, artificial sequence
  Modified bacterial sequence
KEVIEAWDEIDALPNLTLQQWLAFINKLDDDPSQSSELLSEAKKLNDSQ

SEQ ID NO: 275 - protein, 49 aa, artificial sequence
  Modified bacterial sequence
KEVIAAWDEIDKLPNLTIEQWLAFINKLDDDPSQSSELLSEAKKLNDSQ

SEQ ID NO: 276 - protein, 49 aa, artificial sequence
  Modified bacterial sequence
KEVIAAWDEIDKLPNLTLQQWLAFINKLDDDPSQSSELLSEAKKLNDSQ

SEQ ID NO: 277 - protein, 49 aa, artificial sequence
  Modified bacterial sequence
KETIAAWDEIDKLPNLTIEQWLAFINKLDDDPSQSSELLSEAKKLNDSQ

SEQ ID NO: 278 - protein, 49 aa, artificial sequence
  Modified bacterial sequence
KETIEAWNEIDRLPNLTIEQWLAFINKLDDDPSQSSELLSEAKKLNDSQ

SEQ ID NO: 279 - protein, 49 aa, artificial sequence
  Modified bacterial sequence
KEVLEAWREIDALPNLTIQQWLAFINKLDDDPSQSSELLSEAKKLNDSQ

SEQ ID NO: 280 - protein, 49 aa, artificial sequence
  Modified bacterial sequence
KEVIEAWDEIDQLPNLTIEQWLAFINKLDDDPSQSSELLSEAKKLNDSQ

SEQ ID NO: 281 - protein, 49 aa, artificial sequence
  Modified bacterial sequence
KEVLRAWDEIDHLPNLTLEQWLAFINKLDDDPSQSSELLSEAKKLNDSQ

SEQ ID NO: 282 - protein, 49 aa, artificial sequence
  Modified bacterial sequence
KEVLEAWDEIDRLPNLTLNQWLAFINKLDDDPSQSSELLSEAKKLNDSQ

SEQ ID NO: 283 - protein, 49 aa, artificial sequence
  Modified bacterial sequence
KEVLDAWNEIDHLPNLTIEQWLAFINKLDDDPSQSSELLSEAKKLNDSQ

SEQ ID NO: 284 - protein, 49 aa, artificial sequence
  Modified bacterial sequence
KEVIDAWNEIDKLPNLTIEQWLAFINKLDDDPSQSSELLSEAKKLNDSQ

SEQ ID NO: 285 - protein, 49 aa, artificial sequence
  Modified bacterial sequence
KETLEAWDEIDQLPNLTLQQWLAFINKLDDDPSQSSELLSEAKKLNDSQ

SEQ ID NO: 286 - protein, 49 aa, artificial sequence
  Modified bacterial sequence
KEVIEAWNEIDALPNLTLDQWLAFINKLDDDPSQSSELLSEAKKLNDSQ

SEQ ID NO: 287 - protein, 49 aa, artificial sequence
  Modified bacterial sequence
KEVIDAWNEIDRLPNLTLQQWLAFINKLDDDPSQSSELLSEAKKLNDSQ

SEQ ID NO: 288 - protein, 49 aa, artificial sequence
  Modified bacterial sequence
KEVIDAWNEIDQLPNLTLEQWLAFINKLDDDPSQSSELLSEAKKLNDSQ

SEQ ID NO: 289 - protein, 49 aa, artificial sequence
  Modified bacterial sequence
KETIAAWDEIDHLPNLTLEQWLAFINKLDDDPSQSSELLSEAKKLNDSQ

SEQ ID NO: 290 - protein, 49 aa, artificial sequence
  Modified bacterial sequence
KEVLQAWDEIDHLPNLTIQQWLAFINKLSDDPSQSSELLSEAKKLNDSQ

SEQ ID NO: 291 - protein, 49 aa, artificial sequence
  Modified bacterial sequence
KETLHAWAEIDRLPNLTIEQWLAFINKLDDDPSQSSELLSEAKKLNDSQ

SEQ ID NO: 292 - protein, 49 aa, artificial sequence
  Modified bacterial sequence
KEVLEAWNEIDHLPNLTLAQWLAFINKLDDDPSQSSELLSEAKKLNDSQ

SEQ ID NO: 293 - protein, 49 aa, artificial sequence
  Modified bacterial sequence
KEVIEAWDEIDKLPNLTIAQWLAFINKLDDDPSQSSELLSEAKKLNDSQ

SEQ ID NO: 294 - protein, 49 aa, artificial sequence
  Modified bacterial sequence
KEVLDAWDEIDHLPNLTLQQWLAFINKLDDDPSQSSELLSEAKKLNDSQ

SEQ ID NO: 295 - protein, 49 aa, artificial sequence
  Modified bacterial sequence
KETIEAWNEIDKLPNLTLTQWLAFINKLDDDPSQSSELLSEAKKLNDSQ

SEQ ID NO: 296 - protein, 49 aa, artificial sequence
  Modified bacterial sequence
KEVLEAWNEIDLLPNLTIEQWLAFINKLDDDPSQSSELLSEAKKLNDSQ

SEQ ID NO: 297 - protein, 49 aa, artificial sequence
  Modified bacterial sequence
KEVIEAWDEIDHLPNLTIDQWLAFINKLDDDPSQSSELLSEAKKLNDSQ

SEQ ID NO: 298 - protein, 49 aa, artificial sequence
  Modified bacterial sequence
KEVISAWNEIDALPNLTLQQWLAFINKLDDDPSQSSELLSEAKKLNDSQ

SEQ ID NO: 299 - protein, 49 aa, artificial sequence
  Modified bacterial sequence
KEVIAAWNEIDKLPNLTLEQWLAFINKLDDDPSQSSELLSEAKKLNDSQ

SEQ ID NO: 300 - protein, 49 aa, artificial sequence
  Modified bacterial sequence
KETIEAWNEIDSLPNLTLDQWLAFINKLDDDPSQSSELLSEAKKLNDSQ

SEQ ID NO: 301 - protein, 49 aa, artificial sequence
  Modified bacterial sequence
KEVLDAWNEIDQLPNLTLQQWLAFINKLDDDPSQSSELLSEAKKLNDSQ

SEQ ID NO: 302 - protein, 49 aa, artificial sequence
  Modified bacterial sequence
KEVLAAWNEIDHLPNLTIEQWLAFINKLDDDPSQSSELLSEAKKLNDSQ

SEQ ID NO: 303 - protein, 49 aa, artificial sequence
  Modified bacterial sequence
KEVLEAWDEIDHLPNLTITQWLAFINKLDDDPSQSSELLSEAKKLNDSQ

SEQ ID NO: 304 - protein, 49 aa, artificial sequence
  Modified bacterial sequence
KETIDAWNEIDHLPNLTIEQWLAFINKLDDDPSQSSELLSEAKKLNDSQ

SEQ ID NO: 305 - protein, 49 aa, artificial sequence
  Modified bacterial sequence
KEVIEAWNEIDHLPNLTIQQWLAFINKLDDDPSQSSELLSEAKKLNDSQ

SEQ ID NO: 306 - protein, 49 aa, artificial sequence
  Modified bacterial sequence
KEVIQAWNEIDALPNLTISQWLAFINKLDDDPSQSSELLSEAKKLNDSQ

SEQ ID NO: 307 - protein, 49 aa, artificial sequence
  Modified bacterial sequence
KEVIAAWDEIDSLPNLTIEQWLAFINKLDDDPSQSSELLSEAKKLNDSQ

SEQ ID NO: 308 - protein, 49 aa, artificial sequence
  Modified bacterial sequence
KEHIEAWNEIDALPNLTIEQWLAFINKLQDDPSQSSELLSEAKKLNDSQ

SEQ ID NO: 309 - protein, 49 aa, artificial sequence
  Modified bacterial sequence
KEVLEAWNEIDKLPNLTLDQWLAFINKLDDDPSQSSELLSEAKKLNDSQ

SEQ ID NO: 310 - protein, 49 aa, artificial sequence
  Modified bacterial sequence
KEVIDAWNEIDHLPNLTIEQWLAFINKLADDPSQSSELLSEAKKLNDSQ

SEQ ID NO: 311 - protein, 49 aa, artificial sequence
  Modified bacterial sequence
KETIDAWDEIDKLPNLTIEQWLAFINKLDDDPSQSSELLSEAKKLNDSQ

SEQ ID NO: 312 - protein, 49 aa, artificial sequence
  Modified bacterial sequence
KEVIAAWDEIDLLPNLTLQQWLAFINKLADDPSQSSELLSEAKKLNDSQ

SEQ ID NO: 313 - protein, 49 aa, artificial sequence
  Modified bacterial sequence
KEVIHAWDEIDKLPNLTIEQWLAFINKLDDDPSQSSELLSEAKKLNDSQ

SEQ ID NO: 314 - protein, 49 aa, artificial sequence
  Modified bacterial sequence
KEVIAAWNEIDHLPNLTLEQWLAFINKLDDDPSQSSELLSEAKKLNDSQ

SEQ ID NO: 315 - protein, 49 aa, artificial sequence
  Modified bacterial sequence
KETLDAWNEIDKLPNLTLSQWLAFINKLDDDPSQSSELLSEAKKLNDSQ

SEQ ID NO: 316 - protein, 49 aa, artificial sequence
  Modified bacterial sequence
KEVLEAWNEIDALPNLTLEQWLAFINKLDDDPSQSSELLSEAKKLNDSQ

SEQ ID NO: 317 - protein, 49 aa, artificial sequence
  Modified bacterial sequence
KEVIQAWDEIDHLPNLTISQWLAFINKLDDDPSQSSELLSEAKKLNDSQ

SEQ ID NO: 318 - protein, 49 aa, artificial sequence
  Modified bacterial sequence
KEVLQAWDEIDSLPNLTIEQWLAFINKLDDDPSQSSELLSEAKKLNDSQ

SEQ ID NO: 319 - protein, 49 aa, artificial sequence
  Modified bacterial sequence
KETLEAWDEIDHLPNLTIAQWLAFINKLDDDPSQSSELLSEAKKLNDSQ

SEQ ID NO: 320 - protein, 49 aa, artificial sequence
  Modified bacterial sequence
KETIDAWNEIDRLPNLTISQWLAFINKLDDDPSQSSELLSEAKKLNDSQ

SEQ ID NO: 321 - protein, 49 aa, artificial sequence
  Modified bacterial sequence
KEVLDAWHEIDHLPNLTIQQWLAFINKLDDDPSQSSELLSEAKKLNDSQ

SEQ ID NO: 322 - protein, 49 aa, artificial sequence
  Modified bacterial sequence
KEQIRAWDEIDKLPNLTIEQWLAFINKLADDPSQSSELLSEAKKLNDSQ

SEQ ID NO: 323 - protein, 49 aa, artificial sequence
  Modified bacterial sequence
KETLYAWNEIDKLPNLTIEQWLAFIEKLQDDPSQSSELLSEAKKLNDSQ

SEQ ID NO: 324 - protein, 49 aa, artificial sequence
  Modified bacterial sequence
KEVIEAWNEIDALPNLTIDQWLAFINKLDDDPSQSSELLSEAKKLNDSQ

SEQ ID NO: 325 - protein, 49 aa, artificial sequence
  Modified bacterial sequence
KEVLEAWNEIDHLPNLTIQQWLAFINKLDDDPSQSSELLSEAKKLNDSQ

SEQ ID NO: 326 - protein, 49 aa, artificial sequence
  Modified bacterial sequence
KETIEAWDEIDALPNLTIEQWLAFINKLDDDPSQSSELLSEAKKLNDSQ

SEQ ID NO: 327 - protein, 49 aa, artificial sequence
  Modified bacterial sequence
KEVIEAWNEIDHLPNLTLQQWLAFINKLDDDPSQSSELLSEAKKLNDSQ

SEQ ID NO: 328 - protein, 49 aa, artificial sequence
  Modified bacterial sequence
KEVIEAWNEIDKLPNLTIQQWLAFINKLDDDPSQSSELLSEAKKLNDSQ

SEQ ID NO: 329 - protein, 49 aa, artificial sequence
  Modified bacterial sequence
KETLDAWAEIDHLPNLTLDQWLAFINKLDDDPSQSSELLSEAKKLNDSQ

SEQ ID NO: 330 - protein, 49 aa, artificial sequence
  Modified bacterial sequence
KEHIDAWNEIDALPNLTLSQWLAFINKLDDDPSQSSELLSEAKKLNDSQ

SEQ ID NO: 331 - protein, 49 aa, artificial sequence
  Modified bacterial sequence
KEVLDAWNEIDKLPNLTIAQWLAFINKLDDDPSQSSELLSEAKKLNDSQ

SEQ ID NO: 332 - protein, 49 aa, artificial sequence
  Modified bacterial sequence
KEVIEAWTEIDYLPNLTLQQWLAFINKLDDDPSQSSELLSEAKKLNDSQ

SEQ ID NO: 333 - protein, 49 aa, artificial sequence
  Modified bacterial sequence
KETIEAWNEIDHLPNLTIAQWLAFINKLDDDPSQSSELLSEAKKLNDSQ

SEQ ID NO: 334 - protein, 49 aa, artificial sequence
  Modified bacterial sequence
KEVIQAWNEIDKLPNLTLEQWLAFINKLDDDPSQSSELLSEAKKLNDSQ

SEQ ID NO: 335 - protein, 49 aa, artificial sequence
  Modified bacterial sequence
KEVIEAWDEIDHLPNLTIEQWLAFINKLDDDPSQSSELLSEAKKLNDSQ

SEQ ID NO: 336 - protein, 49 aa, artificial sequence
  Modified bacterial sequence
KETIDAWNEIDLLPNLTIEQWLAFINKLDDDPSQSSELLSEAKKLNDSQ

SEQ ID NO: 337 - protein, 49 aa, artificial sequence
  Modified bacterial sequence
KEHIDAWNEIDKLPNLTLDQWLAFINKLDDDPSQSSELLSEAKKLNDSQ

SEQ ID NO: 338 - protein, 49 aa, artificial sequence
  Modified bacterial sequence
KEVVAAWNEIDALPNLTIEQWLAFINKLNDDPSQSSELLSEAKKLNDSQ

SEQ ID NO: 339 - protein, 49 aa, artificial sequence
  Modified bacterial sequence
KEVIEAWNEIDALPNLTLAQWLAFINKLDDDPSQSSELLSEAKKLNDSQ

SEQ ID NO: 340 - protein, 49 aa, artificial sequence
  Modified bacterial sequence
KEVLQAWDEIDRLPNLTLDQWLAFINKLDDDPSQSSELLSEAKKLNDSQ

SEQ ID NO: 341 - protein, 49 aa, artificial sequence
  Modified bacterial sequence
KEVIDAWDEIDHLPNLTIEQWLAFINKLSDDPSQSSELLSEAKKLNDSQ

SEQ ID NO: 342 - protein, 49 aa, artificial sequence
  Modified bacterial sequence
KEVVEAWNEIDQLPNLTIEQWLAFINKLDDDPSQSSELLSEAKKLNDSQ

SEQ ID NO: 343 - protein, 49 aa, artificial sequence
  Modified bacterial sequence
KEVIQAWNEIDALPNLTIEQWLAFINKLDDDPSQSSELLSEAKKLNDSQ

SEQ ID NO: 344 - protein, 49 aa, artificial sequence
  Modified bacterial sequence
KEVIQAWDEIDKLPNLTIDQWLAFINKLADDPSQSSELLSEAKKLNDSQ

SEQ ID NO: 345 - protein, 49 aa, artificial sequence
  Modified bacterial sequence
KEVVAAWDEIDALPNLTLTQWLAFINKLDDDPSQSSELLSEAKKLNDSQ

SEQ ID NO: 346 - protein, 49 aa, artificial sequence
  Modified bacterial sequence
KEVIQAWNEIDGLPNLTLSQWLAFINKLDDDPSQSSELLSEAKKLNDSQ

SEQ ID NO: 347 - protein, 49 aa, artificial sequence
  Modified bacterial sequence
KETIEAWDEIDALPNLTITQWLAFINKLDDDPSQSSELLSEAKKLNDSQ

SEQ ID NO: 348 - protein, 49 aa, artificial sequence
  Modified bacterial sequence
KEVIDAWNEIDHLPNLTIQQWLAFINKLADDPSQSSELLSEAKKLNDSQ

SEQ ID NO: 349 - protein, 49 aa, artificial sequence
  Modified bacterial sequence
KETIEAWNEIDALPNLTLDQWLAFINKLEDDPSQSSELLSEAKKLNDSQ

SEQ ID NO: 350 - protein, 49 aa, artificial sequence
  Modified bacterial sequence
KEHIHAWNEIDELPNLTIEQWLAFINKLADDPSQSSELLSEAKKLNDSQ

SEQ ID NO: 351 - protein, 49 aa, artificial sequence
  Modified bacterial sequence
KEVIDAWDEIDHLPNLTIDQWLAFINKLSDDPSQSSELLSEAKKLNDSQ

SEQ ID NO: 352 - protein, 49 aa, artificial sequence
  Modified bacterial sequence
KEVIDANDEIDALPNLTIAQWLAFINKLHDDPSQSSELLSEAKKLNDSQ

SEQ ID NO: 353 - protein, 49 aa, artificial sequence
  Modified bacterial sequence
KETIEAWDEIDKLPNLTIEQWLAFINKLDDDPSQSSELLSEAKKLNDSQ

SEQ ID NO: 354 - protein, 49 aa, artificial sequence
  Modified bacterial sequence
KEVLLAWDEIDHLPNLTLEQWLAFINKLDDDPSQSSELLSEAKKLNDSQ

SEQ ID NO: 355 - protein, 49 aa, artificial sequence
  Modified bacterial sequence
KEHIDAWNEIDGLPNLTLEQWLAFINKLDDDPSQSSELLSEAKKLNDSQ

SEQ ID NO: 356 - protein, 49 aa, artificial sequence
  Modified bacterial sequence
KEVIEAWSEIDALPNLTIDQWLAFINKLADDPSQSSELLSEAKKLNDSQ

SEQ ID NO: 357 - protein, 49 aa, artificial sequence
  Modified bacterial sequence
KEQLNAWAEIDALPNLTIEQWLAFINKLDDDPSQSSELLSEAKKLNDSQ

SEQ ID NO: 358 - protein, 49 aa, artificial sequence
  Modified bacterial sequence
KEVIDAWNEIDALPNLTIAQWLAFINKLDDDPSQSSELLSEAKKLNDSQ

SEQ ID NO: 359 - protein, 49 aa, artificial sequence
  Modified bacterial sequence
KETIDAWNEIDQLPNLTIEQWLAFINKLDDDPSQSSELLSEAKKLNDSQ

SEQ ID NO: 360 - protein, 49 aa, artificial sequence
  Modified bacterial sequence
KEVIEAWDEIDKLPNLTLAQWLAFINKLDDDPSQSSELLSEAKKLNDSQ

SEQ ID NO: 361 - protein, 49 aa, artificial sequence
  Modified bacterial sequence
KEVLYAWAEIDHLPNLTIEQWLAFINKLDDDPSQSSELLSEAKKLNDSQ

SEQ ID NO: 362 - protein, 49 aa, artificial sequence
  Modified bacterial sequence
KEQIDAWNEIDRLPNLTIQQWLAFINKLDDDPSQSSELLSEAKKLNDSQ

SEQ ID NO: 363 - protein, 49 aa, artificial sequence
  Modified bacterial sequence
KEVLAAWDEIDRLPNLTIEQWLAFINKLDDDPSQSSELLSEAKKLNDSQ

SEQ ID NO: 364 - protein, 49 aa, artificial sequence
  Modified bacterial sequence
KEVIEAWDEIDHLPNLTLHQWLAFINKLDDDPSQSSELLSEAKKLNDSQ

SEQ ID NO: 365 - protein, 49 aa, artificial sequence
  Modified bacterial sequence
KEVIEAWNEIDKLPNLTLQQWLAFINKLDDDPSQSSELLSEAKKLNDSQ

SEQ ID NO: 366 - protein, 49 aa, artificial sequence
  Modified bacterial sequence
KEVIDANDEIDALPNLTIEQWLAFINKLHDDPSQSSELLSEAKKLNDSQ

SEQ ID NO: 367 - protein, 49 aa, artificial sequence
  Modified bacterial sequence
KEVIAAWDEIDALPNLTIEQWLAFINKLDDDPSQSSELLSEAKKLNDSQ

SEQ ID NO: 368 - protein, 49 aa, artificial sequence
  Modified bacterial sequence
KEVIEAWTEIDQLPNLTLDQWLAFINKLDDDPSQSSELLSEAKKLNDSQ

SEQ ID NO: 369 - protein, 49 aa, artificial sequence
  Modified bacterial sequence
KEVINAWNEIDALPNLTLQQWLAFINKLDDDPSQSSELLSEAKKLNDSQ

SEQ ID NO: 370 - protein, 49 aa, artificial sequence
  Modified bacterial sequence
KEHIEAWDEIDHLPNLTIDQWLAFINKLADDPSQSSELLSEAKKLNDSQ

SEQ ID NO: 371 - protein, 49 aa, artificial sequence
  Modified bacterial sequence
KEHLEAWREIDALPNLTIEQWLAFINKLDDDPSQSSELLSEAKKLNDSQ

SEQ ID NO: 372 - protein, 49 aa, artificial sequence
  Modified bacterial sequence
KEVLDAWNEIDKLPNLTLQQWLAFINKLDDDPSQSSELLSEAKKLNDSQ

SEQ ID NO: 373 - protein, 49 aa, artificial sequence
  Modified bacterial sequence
KEVIAAWDEIDHLPNLTIQQWLAFINKLDDDPSQSSELLSEAKKLNDSQ

SEQ ID NO: 374 - protein, 49 aa, artificial sequence
  Modified bacterial sequence
KEVIQAWNEIDALPNLTLEQWLAFINKLDDDPSQSSELLSEAKKLNDSQ

SEQ ID NO: 375 - protein, 49 aa, artificial sequence
  Modified bacterial sequence
KEVIDAWNEIDHLPNLTIAQWLAFINKLDDDPSQSSELLSEAKKLNDSQ

SEQ ID NO: 376 - protein, 49 aa, artificial sequence
  Modified bacterial sequence
KEQLDAWDEIDHLPNLTIDQWLAFINKLSDDPSQSSELLSEAKKLNDSQ

SEQ ID NO: 377 - protein, 49 aa, artificial sequence
  Modified bacterial sequence
KEVLNAWDEIDKLPNLTIEQWLAFINKLDDDPSQSSELLSEAKKLNDSQ

SEQ ID NO: 378 - protein, 49 aa, artificial sequence
  Modified bacterial sequence
KEVLEAWNEIDHLPNLTIDQWLAFINKLDDDPSQSSELLSEAKKLNDSQ

SEQ ID NO: 379 - protein, 49 aa, artificial sequence
  Modified bacterial sequence
KEVLLAWDEIDRLPNLTIDQWLAFINKLADDPSQSSELLSEAKKLNDSQ

SEQ ID NO: 380 - protein, 49 aa, artificial sequence
  Modified bacterial sequence
KEVIAAWNEIDQLPNLTLDQWLAFINKLDDDPSQSSELLSEAKKLNDSQ

SEQ ID NO: 381 - protein, 49 aa, artificial sequence
  Modified bacterial sequence
KETLLAWDEIDALPNLTIEQWLAFINKLDDDPSQSSELLSEAKKLNDSQ

SEQ ID NO: 382 - protein, 49 aa, artificial sequence
  Modified bacterial sequence
KEVIDAWNEIDTLPNLTLEQWLAFINKLDDDPSQSSELLSEAKKLNDSQ

SEQ ID NO: 383 - protein, 49 aa, artificial sequence
  Modified bacterial sequence
KEVLHAWNEIDHLPNLTLNQWLAFINKLQDDPSQSSELLSEAKKLNDSQ

SEQ ID NO: 384 - protein, 49 aa, artificial sequence
  Modified bacterial sequence
KEVIQAWNEIDALPNLTIAQWLAFINKLDDDPSQSSELLSEAKKLNDSQ

SEQ ID NO: 385 - protein, 49 aa, artificial sequence
  Modified bacterial sequence
KETVDAWNEIDALPNLTIEQWLAFINKLDDDPSQSSELLSEAKKLNDSQ

SEQ ID NO: 386 - protein, 49 aa, artificial sequence
  Modified bacterial sequence
KEVIQAWDEIDHLPNLTIDQWLAFINKLDDDPSQSSELLSEAKKLNDSQ

SEQ ID NO: 387 - protein, 49 aa, artificial sequence
  Modified bacterial sequence
KEVLDAWNEIDQLPNLTIQQWLAFINKLDDDPSQSSELLSEAKKLNDSQ

SEQ ID NO: 388 - protein, 49 aa, artificial sequence
  Modified bacterial sequence
KETIEAWNEIDALPNLTLDQWLAFINKLDDDPSQSSELLSEAKKLNDSQ

SEQ ID NO: 389 - protein, 49 aa, artificial sequence
  Modified bacterial sequence
KEVIEAWDEIDALPNLTIDQWLAFINKLDDDPSQSSELLSEAKKLNDSQ

SEQ ID NO: 390 - protein, 49 aa, artificial sequence
  Modified bacterial sequence
KEVIEAWNEIDQLPNLTIQQWLAFINKLDDDPSQSSELLSEAKKLNDSQ

SEQ ID NO: 391 - protein, 49 aa, artificial sequence
  Modified bacterial sequence
KEVIEAWTEIDHLPNLTIEQWLAFINKLDDDPSQSSELLSEAKKLNDSQ

SEQ ID NO: 392 - protein, 49 aa, artificial sequence
  Modified bacterial sequence
KEVIQAWNEIDHLPNLTLQQWLAFINKLEDDPSQSSELLSEAKKLNDSQ

SEQ ID NO: 393 - protein, 49 aa, artificial sequence
  Modified bacterial sequence
KEVIQANNEIDQLPNLTIEQWLAFINKLHDDPSQSSELLSEAKKLNDSQ

SEQ ID NO: 394 - protein, 49 aa, artificial sequence
  Modified bacterial sequence
KEVLHAWSEIDKLPNLTIEQWLAFINKLDDDPSQSSELLSEAKKLNDSQ

SEQ ID NO: 395 - protein, 49 aa, artificial sequence
  Modified bacterial sequence
KETIQAWDEIDKLPNLTLDQWLAFINKLSDDPSQSSELLSEAKKLNDSQ

SEQ ID NO: 396 - protein, 49 aa, artificial sequence
  Modified bacterial sequence
KETLRAWDEIDKLPNLTIQQWLAFINKLADDPSQSSELLSEAKKLNDSQ

SEQ ID NO: 397 - protein, 49 aa, artificial sequence
  Modified bacterial sequence
KEVIDAWNEIDHLPNLTIEQWLAFINKLEDDPSQSSELLSEAKKLNDSQ

SEQ ID NO: 398 - protein, 49 aa, artificial sequence
  Modified bacterial sequence
KEVIDAWNEIDHLPNLTLQQWLAFINKLADDPSQSSELLSEAKKLNDSQ

SEQ ID NO: 399 - protein, 49 aa, artificial sequence
  Modified bacterial sequence
KETIDAWNEIDALPNLTLDQWLAFINKLDDDPSQSSELLSEAKKLNDSQ

SEQ ID NO: 400 - protein, 49 aa, artificial sequence
  Modified bacterial sequence
KEVIEAWNEIDQLPNLTIEQWLAFINKLDDDPSQSSELLSEAKKLNDSQ

SEQ ID NO: 401 - protein, 49 aa, artificial sequence
  Modified bacterial sequence
KEVIRAWDEIDQLPNLTLSQWLAFINKLDDDPSQSSELLSEAKKLNDSQ

SEQ ID NO: 402 - protein, 49 aa, artificial sequence
  Modified bacterial sequence
KEVIEAWNEIDRLPNLTIHQWLAFINKLDDDPSQSSELLSEAKKLNDSQ

SEQ ID NO: 403 - protein, 49 aa, artificial sequence
  Modified bacterial sequence
KETIEAWNEIDQLPNLTIEQWLAFINKLDDDPSQSSELLSEAKKLNDSQ

SEQ ID NO: 404 - protein, 49 aa, artificial sequence
  Modified bacterial sequence
KEVLTAWAEIDALPNLTLSQWLAFINKLDDDPSQSSELLSEAKKLNDSQ

SEQ ID NO: 405 - protein, 49 aa, artificial sequence
  Modified bacterial sequence
KEVIEAWDEIDKLPNLTVDQWLAFINKLDDDPSQSSELLSEAKKLNDSQ

SEQ ID NO: 406 - protein, 49 aa, artificial sequence
  Modified bacterial sequence
KEVIDAWNEIDHLPNLTLTQWLAFINKLDDDPSQSSELLSEAKKLNDSQ

SEQ ID NO: 407 - protein, 49 aa, artificial sequence
  Modified bacterial sequence
KEVIEAWNEIDQLPNLTLDQWLAFINKLDDDPSQSSELLSEAKKLNDSQ

SEQ ID NO: 408 - protein, 49 aa, artificial sequence
  Modified bacterial sequence
KETLQAWDEIDHLPNLTLNQWLAFINKLDDDPSQSSELLSEAKKLNDSQ

SEQ ID NO: 409 - protein, 49 aa, artificial sequence
  Modified bacterial sequence
KEVIDAWNEIDHLPNLTIEQWLAFINKLDDDPSQSSELLSEAKKLNDSQ

SEQ ID NO: 410 - protein, 49 aa, artificial sequence
  Modified bacterial sequence
KEVIEAWNEIDLLPNLTLSQWLAFINKLDDDPSQSSELLSEAKKLNDSQ

SEQ ID NO: 411 - protein, 49 aa, artificial sequence
  Modified bacterial sequence
KEVIDAWDEIDRLPNLTLKQWLAFINKLDDDPSQSSELLSEAKKLNDSQ

SEQ ID NO: 412 - protein, 49 aa, artificial sequence
  Modified bacterial sequence
KETLHAWDEIDKLPNLTIEQWLAFINKLDDDPSQSSELLSEAKKLNDSQ

SEQ ID NO: 413 - protein, 49 aa, artificial sequence
  Modified bacterial sequence
KEVIKAWDEIDHLPNLTLNQWLAFINKLDDDPSQSSELLSEAKKLNDSQ

SEQ ID NO: 414 - protein, 49 aa, artificial sequence
  Modified bacterial sequence
KEVIEAWNEIDHLPNLTLAQWLAFINKLDDDPSQSSELLSEAKKLNDSQ

SEQ ID NO: 415 - protein, 49 aa, artificial sequence
  Modified bacterial sequence
KEVIQAWNEIDHLPNLTIDQWLAFITKLEDDPSQSSELLSEAKKLNDSQ

SEQ ID NO: 416 - protein, 49 aa, artificial sequence
  Modified bacterial sequence
KEVIEAWNEIDRLPNLTIKQWLAFINKLDDDPSQSSELLSEAKKLNDSQ

SEQ ID NO: 417 - protein, 49 aa, artificial sequence
  Modified bacterial sequence
KEVIEAWNEIDSLPNLTLQQWLAFINKLDDDPSQSSELLSEAKKLNDSQ

SEQ ID NO: 418 - protein, 49 aa, artificial sequence
  Modified bacterial sequence
KETIDAWNEIDKLPNLTIEQWLAFINKLDDDPSQSSELLSEAKKLNDSQ

SEQ ID NO: 419 - protein, 49 aa, artificial sequence
  Modified bacterial sequence
KEVLEAWAEIDALPNLTIAQWLAFINKLDDDPSQSSELLSEAKKLNDSQ

SEQ ID NO: 420 - protein, 49 aa, artificial sequence
  Modified bacterial sequence
KETIDAWNEIDRLPNLTIEQWLAFINKLDDDPSQSSELLSEAKKLNDSQ

SEQ ID NO: 421 - protein, 49 aa, artificial sequence
  Modified bacterial sequence
KETLKAWDEIDRLPNLTLEQWLAFINKLDDDPSQSSELLSEAKKLNDSQ

SEQ ID NO: 422 - protein, 49 aa, artificial sequence
  Modified bacterial sequence
KETIAAWNEIDALPNLTLQQWLAFINKLDDDPSQSSELLSEAKKLNDSQ

SEQ ID NO: 423 - protein, 49 aa, artificial sequence
  Modified bacterial sequence
KEVLQAWNEIDHLPNLTIQQWLAFINKLDDDPSQSSELLSEAKKLNDSQ

SEQ ID NO: 424 - protein, 49 aa, artificial sequence
  Modified bacterial sequence
KEVIEAWSEIDHLPNLTLQQWLAFINKLDDDPSQSSELLSEAKKLNDSQ

SEQ ID NO: 425 - protein, 49 aa, artificial sequence
  Modified bacterial sequence
KEVIDAWNEIDGLPNLTIEQWLAFINKLDDDPSQSSELLSEAKKLNDSQ

SEQ ID NO: 426 - protein, 49 aa, artificial sequence
  Modified bacterial sequence
KEVIHAWNEIDHLPNLTLNQWLAFINKLEDDPSQSSELLSEAKKLNDSQ

SEQ ID NO: 427 - protein, 49 aa, artificial sequence
  Modified bacterial sequence
KEVLDAWNEIDSLPNLTLDQWLAFINKLDDDPSQSSELLSEAKKLNDSQ

SEQ ID NO: 428 - protein, 49 aa, artificial sequence
  Modified bacterial sequence
KEQIEAWNEIDRLPNLTLEQWLAFINKLDDDPSQSSELLSEAKKLNDSQ

SEQ ID NO: 429 - protein, 49 aa, artificial sequence
  Modified bacterial sequence
KEVVDAWNEIDALPNLTLQQWLAFINKLDDDPSQSSELLSEAKKLNDSQ

SEQ ID NO: 430 - protein, 49 aa, artificial sequence
  Modified bacterial sequence
KEVIEAWNEIDKLPNLTIEQWLAFINKLDDDPSQSSELLSEAKKLNDSQ

SEQ ID NO: 431 - protein, 49 aa, artificial sequence
  Modified bacterial sequence
KEVIEANDEIDRLPNLTIEQWLAFINKLHDDPSQSSELLSEAKKLNDSQ

SEQ ID NO: 432 - protein, 49 aa, artificial sequence
  Modified bacterial sequence
KETLQAWDEIDKLPNLTIEQWLAFINKLDDDPSQSSELLSEAKKLNDSQ

SEQ ID NO: 433 - protein, 49 aa, artificial sequence
  Modified bacterial sequence
KEVIEAWDEIDHLPNLTIDQWLAFINKLADDPSQSSELLSEAKKLNDSQ

SEQ ID NO: 434 - protein, 49 aa, artificial sequence
  Modified bacterial sequence
KETIDAWNEIDHLPNLTLQQWLAFINKLADDPSQSSELLSEAKKLNDSQ

SEQ ID NO: 435 - protein, 49 aa, artificial sequence
  Modified bacterial sequence
KEVIDAWDEIDKLPNLTIEQWLAFINKLDDDPSQSSELLSEAKKLNDSQ

SEQ ID NO: 436 - protein, 49 aa, artificial sequence
  Modified bacterial sequence
KEVIEAWNEIDKLPNLTLAQWLAFINKLDDDPSQSSELLSEAKKLNDSQ

SEQ ID NO: 437 - protein, 49 aa, artificial sequence
  Modified bacterial sequence
KEVLQAWDEIDKLPNLTIQQWLAFINKLDDDPSQSSELLSEAKKLNDSQ

SEQ ID NO: 438 - protein, 49 aa, artificial sequence
  Modified bacterial sequence
KEVIAAWNEIDGLPNLTLQQWLAFINKLDDDPSQSSELLSEAKKLNDSQ

SEQ ID NO: 439 - protein, 49 aa, artificial sequence
  Modified bacterial sequence
KETLNAWNEIDALPNLTLQQWLAFINKLDDDPSQSSELLSEAKKLNDSQ

SEQ ID NO: 440 - protein, 49 aa, artificial sequence
  Modified bacterial sequence
KEVLSAWNEIDQLPNLTLEQWLAFINKLDDDPSQSSELLSEAKKLNDSQ

SEQ ID NO: 441 - protein, 49 aa, artificial sequence
  Modified bacterial sequence
KETLEAWDEIDHLPNLTLHQWLAFINKLDDDPSQSSELLSEAKKLNDSQ

SEQ ID NO: 442 - protein, 49 aa, artificial sequence
  Modified bacterial sequence
KEQIEAWNEIDHLPNLTLQQWLAFINKLADDPSQSSELLSEAKKLNDSQ

SEQ ID NO: 443 - protein, 49 aa, artificial sequence
  Modified bacterial sequence
KEVVEAWDEIDKLPNLTIEQWLAFINKLDDDPSQSSELLSEAKKLNDSQ

SEQ ID NO: 444 - protein, 49 aa, artificial sequence
  Modified bacterial sequence
KEVLEAWNEIDELPNLTIEQWLAFINKLDDDPSQSSELLSEAKKLNDSQ

SEQ ID NO: 445 - protein, 49 aa, artificial sequence
  Modified bacterial sequence
KEVIDAWNEIDQLPNLTLQQWLAFINKLDDDPSQSSELLSEAKKLNDSQ

SEQ ID NO: 446 - protein, 49 aa, artificial sequence
  Modified bacterial sequence
KETIDAWDEIDKLPNLTLSQWLAFINKLDDDPSQSSELLSEAKKLNDSQ

SEQ ID NO: 447 - protein, 49 aa, artificial sequence
  Modified bacterial sequence
KETIDAWNEIDQLPNLTLQQWLAFINKLDDDPSQSSELLSEAKKLNDSQ

SEQ ID NO: 448 - protein, 49 aa, artificial sequence
  Modified bacterial sequence
KEVIQAWDEIDALPNLTLNQWLAFINKLDDDPSQSSELLSEAKKLNDSQ

SEQ ID NO: 449 - protein, 49 aa, artificial sequence
  Modified bacterial sequence
KEVLDAWAEIDQLPNLTLQQWLAFINKLDDDPSQSSELLSEAKKLNDSQ

SEQ ID NO: 450 - protein, 49 aa, artificial sequence
  Modified bacterial sequence
KEHIAAWDEIDALPNLTIEQWLAFINKLDDDPSQSSELLSEAKKLNDSQ

SEQ ID NO: 451 - protein, 49 aa, artificial sequence
  Modified bacterial sequence
KEVIRAWDEIDALPNLTIEQWLAFINKLDDDPSQSSELLSEAKKLNDSQ

SEQ ID NO: 452 - protein, 49 aa, artificial sequence
  Modified bacterial sequence
KEVIDAWDEIDALPNLTIDQWLAFINKLADDPSQSSELLSEAKKLNDSQ

SEQ ID NO: 453 - protein, 49 aa, artificial sequence
  Modified bacterial sequence
KEVIDAWNEIDRLPNLTIQQWLAFINKLDDDPSQSSELLSEAKKLNDSQ

SEQ ID NO: 454 - protein, 49 aa, artificial sequence
  Modified bacterial sequence
KEVITAWNEIDHLPNLTLSQWLAFINKLDDDPSQSSELLSEAKKLNDSQ

SEQ ID NO: 455 - protein, 49 aa, artificial sequence
  Modified bacterial sequence
KEVIDAWNEIDALPNLTIHQWLAFINKLDDDPSQSSELLSEAKKLNDSQ

SEQ ID NO: 456 - protein, 49 aa, artificial sequence
  Modified bacterial sequence
KEQLKAWDEIDKLPNLTIEQWLAFIEKLQDDPSQSSELLSEAKKLNDSQ

SEQ ID NO: 457 - protein, 49 aa, artificial sequence
  Modified bacterial sequence
KEHIDAWTEIDHLPNLTIEQWLAFINKLDDDPSQSSELLSEAKKLNDSQ

SEQ ID NO: 458 - protein, 49 aa, artificial sequence
  Modified bacterial sequence
KEQLRAWDEIDKLPNLTIEQWLAFINKLQDDPSQSSELLSEAKKLNDSQ

SEQ ID NO: 459 - protein, 49 aa, artificial sequence
  Modified bacterial sequence
KEVLEAWREIDSLPNLTIAQWLAFINKLDDDPSQSSELLSEAKKLNDSQ

SEQ ID NO: 460 - protein, 49 aa, artificial sequence
  Modified bacterial sequence
KEVIQAWNEIDKLPNLTIEQWLAFINKLDDDPSQSSELLSEAKKLNDSQ

SEQ ID NO: 461 - protein, 49 aa, artificial sequence
  Modified bacterial sequence
KEHVEAWNEIDQLPNLTIEQWLAFINKLADDPSQSSELLSEAKKLNDSQ

SEQ ID NO: 462 - protein, 49 aa, artificial sequence
  Modified bacterial sequence
KEVIDAWDEIDALPNLTIDQWLAFINKLSDDPSQSSELLSEAKKLNDSQ

SEQ ID NO: 463 - protein, 49 aa, artificial sequence
  Modified bacterial sequence
KEVIEAWNEIDHLPNLTIEQWLAFINKLDDDPSQSSELLSEAKKLNDSQ

SEQ ID NO: 464 - protein, 49 aa, artificial sequence
  Modified bacterial sequence
KEVLQAWDEIDKLPNLTIEQWLAFINKLSDDPSQSSELLSEAKKLNDSQ

SEQ ID NO: 465 - protein, 49 aa, artificial sequence
  Modified bacterial sequence
KEVIKAWNEIDSLPNLTIEQWLAFINKLDDDPSQSSELLSEAKKLNDSQ

SEQ ID NO: 466 - protein, 49 aa, artificial sequence
  Modified bacterial sequence
KEVLEAWHEIDLLPNLTIQQWLAFINKLDDDPSQSSELLSEAKKLNDSQ

SEQ ID NO: 467 - protein, 49 aa, artificial sequence
  Modified bacterial sequence
KEVLEAWTEIDRLPNLTLDQWLAFINKLDDDPSQSSELLSEAKKLNDSQ

SEQ ID NO: 468 - protein, 49 aa, artificial sequence
  Modified bacterial sequence
KEQLYAWNEIDHLPNLTIEQWLAFIEKLQDDPSQSSELLSEAKKLNDSQ

SEQ ID NO: 469 - protein, 49 aa, artificial sequence
  Modified bacterial sequence
KEVLNAWDEIDKLPNLTIKQWLAFINKLDDDPSQSSELLSEAKKLNDSQ

SEQ ID NO: 470 - protein, 49 aa, artificial sequence
  Modified bacterial sequence
KEVIRAWDEIDKLPNLTVEQWLAFINKLDDDPSQSSELLSEAKKLNDSQ

SEQ ID NO: 471 - protein, 49 aa, artificial sequence
  Modified bacterial sequence
KEVVQAWDEIDQLPNLTLEQWLAFINKLDDDPSQSSELLSEAKKLNDSQ

SEQ ID NO: 472 - protein, 49 aa, artificial sequence
  Modified bacterial sequence
KEVIRAWDEIDQLPNLTLEQWLAFINKLDDDPSQSSELLSEAKKLNDSQ

SEQ ID NO: 473 - protein, 49 aa, artificial sequence
  Modified bacterial sequence
KETIDAWNEIDHLPNLTLDQWLAFINKLDDDPSQSSELLSEAKKLNDSQ

SEQ ID NO: 474 - protein, 49 aa, artificial sequence
  Modified bacterial sequence
KEVVAAWTEIDLLPNLTLDQWLAFINKLEDDPSQSSELLSEAKKLNDSQ

SEQ ID NO: 475 - protein, 49 aa, artificial sequence
  Modified bacterial sequence
KEVVAAWDEIDALPNLTIEQWLAFINKLSDDPSQSSELLSEAKKLNDSQ

SEQ ID NO: 476 - protein, 49 aa, artificial sequence
  Modified bacterial sequence
KETLEAWREIDSLPNLTLEQWLAFINKLDDDPSQSSELLSEAKKLNDSQ

SEQ ID NO: 477 - protein, 49 aa, artificial sequence
  Modified bacterial sequence
KEVIKAWNEIDHLPNLTLDQWLAFINKLDDDPSQSSELLSEAKKLNDSQ

SEQ ID NO: 478 - protein, 49 aa, artificial sequence
  Modified bacterial sequence
KEVLEAWTEIDKLPNLTIDQWLAFINKLDDDPSQSSELLSEAKKLNDSQ

SEQ ID NO: 479 - protein, 49 aa, artificial sequence
  Modified bacterial sequence
KETLEAWDEIDKLPNLTIDQWLAFINKLDDDPSQSSELLSEAKKLNDSQ

SEQ ID NO: 480 - protein, 49 aa, artificial sequence
  Modified bacterial sequence
KEVIEAWNEIDKLPNLTIDQWLAFINKLDDDPSQSSELLSEAKKLNDSQ

SEQ ID NO: 481 - protein, 49 aa, artificial sequence
  Modified bacterial sequence
KETIDAWNEIDKLPNLTLEQWLAFINKLDDDPSQSSELLSEAKKLNDSQ

SEQ ID NO: 482 - protein, 49 aa, artificial sequence
  Modified bacterial sequence
KETLDAWDEIDALPNLTIDQWLAFINKLEDDPSQSSELLSEAKKLNDSQ

SEQ ID NO: 483 - protein, 49 aa, artificial sequence
  Modified bacterial sequence
KEVLSAWNEIDHLPNLTIQQWLAFINKLDDDPSQSSELLSEAKKLNDSQ

SEQ ID NO: 484 - protein, 49 aa, artificial sequence
  Modified bacterial sequence
KEVIQANDEIDKLPNLTIEQWLAFIHKLHDDPSQSSELLSEAKKLNDSQ

SEQ ID NO: 485 - protein, 49 aa, artificial sequence
  Modified bacterial sequence
KEHLDAWDEIDHLPNLTIQQWLAFINKLADDPSQSSELLSEAKKLNDSQ

SEQ ID NO: 486 - protein, 49 aa, artificial sequence
  Modified bacterial sequence
KEVIQAWNEIDQLPNLTIEQWLAFINKLDDDPSQSSELLSEAKKLNDSQ

SEQ ID NO: 487 - protein, 49 aa, artificial sequence
  Modified bacterial sequence
KEVIEAWNEIDYLPNLTIAQWIAFINKLDDDPSQSSELLSEAKKLNDSQ

SEQ ID NO: 488 - protein, 49 aa, artificial sequence
  Modified bacterial sequence
KETIQAWDEIDRLPNLTLQQWLAFINKLDDDPSQSSELLSEAKKLNDSQ

SEQ ID NO: 489 - protein, 49 aa, artificial sequence
  Modified bacterial sequence
KETIQAWDEIDKLPNLTIEQWLAFINKLDDDPSQSSELLSEAKKLNDSQ

SEQ ID NO: 490 - protein, 49 aa, artificial sequence
  Modified bacterial sequence
KETLDAWAEIDHLPNLTIEQWLAFINKLDDDPSQSSELLSEAKKLNDSQ

SEQ ID NO: 491 - protein, 49 aa, artificial sequence
  Modified bacterial sequence
KEVIEAWDEIDKLPNLTLNQWLAFINKLDDDPSQSSELLSEAKKLNDSQ

SEQ ID NO: 492 - protein, 49 aa, artificial sequence
  Modified bacterial sequence
KEVLDAWNEIDQLPNLTIEQWLAFINKLDDDPSQSSELLSEAKKLNDSQ

SEQ ID NO: 493 - protein, 49 aa, artificial sequence
  Modified bacterial sequence
KEVLHAWNEIDHLPNLTIEQWLAFIEKLEDDPSQSSELLSEAKKLNDSQ

SEQ ID NO: 494 - protein, 49 aa, artificial sequence
  Modified bacterial sequence
KEVIEAWQEIDKLPNLTIDQWLAFINKLDDDPSQSSELLSEAKKLNDSQ

SEQ ID NO: 495 - protein, 49 aa, artificial sequence
  Modified bacterial sequence
KEVVDAWNEIDQLPNLTIEQWLAFINKLDDDPSQSSELLSEAKKLNDSQ

SEQ ID NO: 496 - protein, 49 aa, artificial sequence
  Modified bacterial sequence
KEQIEAWNEIDALPNLTIEQWLAFINKLADDPSQSSELLSEAKKLNDSQ

SEQ ID NO: 497 - protein, 58 aa, artificial sequence
  Modified bacterial sequence
VDAKYAKEVLEAWDEIDRLPNLTIEQWLAFINKLDDDPSQSSELLSEAKKLNDSQAPK

SEQ ID NO: 498 - protein, 58 aa, artificial sequence
  Modified bacterial sequence
VDAKYAKEVLEAWNEIDRLPNLTIEQWLAFINKLDDDPSQSSELLSEAKKLNDSQAPK

SEQ ID NO: 499 - protein, 58 aa, artificial sequence
  Modified bacterial sequence
VDAKYAKEVIEAWNEIDRLPNLTIEQWLAFINKLDDDPSQSSELLSEAKKLNDSQAPK

SEQ ID NO: 500 - protein, 58 aa, artificial sequence
  Modified bacterial sequence
VDAKYAKEVLEAWDEIDRLPNLTLDQWLAFINKLDDDPSQSSELLSEAKKLNDSQAPK

SEQ ID NO: 501 - protein, 58 aa, artificial sequence
  Modified bacterial sequence
VDAKYAKEVLDAWDEIDALPNLTLEQWLAFINKLDDDPSQSSELLSEAKKLNDSQAPK

SEQ ID NO: 502 - protein, 58 aa, artificial sequence
  Modified bacterial sequence
VDAKYAKEVIDAWDEIDRLPNLTLDQWLAFINKLDDDPSQSSELLSEAKKLNDSQAPK

SEQ ID NO: 503 - protein, 58 aa, artificial sequence
  Modified bacterial sequence
VDAKYAKETLEAWDEIDRLPNLTIEQWLAFINKLDDDPSQSSELLSEAKKLNDSQAPK

SEQ ID NO: 504 - protein, 58 aa, artificial sequence
  Modified bacterial sequence
VDAKYAKEVIDAWNEIDALPNLTLDQWLAFINKLDDDPSQSSELLSEAKKLNDSQAPK

SEQ ID NO: 505 - protein, 58 aa, artificial sequence
  Modified bacterial sequence
VDAKYAKEVLDAWDEIDKLPNLTIDQWLAFINKLDDDPSQSSELLSEAKKLNDSQAPK

SEQ ID NO: 506 - protein, 58 aa, artificial sequence
  Modified bacterial sequence
VDAKYAKEVLEAWDEIDHLPNLTLDQWLAFINKLDDDPSQSSELLSEAKKLNDSQAPK

SEQ ID NO: 507 - protein, 58 aa, artificial sequence
  Modified bacterial sequence
VDAKYAKEVLEAWDEIDALPNLTIEQWLAFINKLDDDPSQSSELLSEAKKLNDSQAPK

SEQ ID NO: 508 - protein, 58 aa, artificial sequence
  Modified bacterial sequence
VDAKYAKEVLDAWDEIDKLPNLTLEQWLAFINKLDDDPSQSSELLSEAKKLNDSQAPK

SEQ ID NO: 509 - protein, 58 aa, artificial sequence
  Modified bacterial sequence
VDAKYAKETITAWDEIDKLPNLTIEQWLAFIGKLEDDPSQSSELLAEAKKLNDAQAPK

SEQ ID NO: 510 - protein, 58 aa, artificial sequence
  Modified bacterial sequence
VDNKFNKESMKAWDEIDRLPNLNINQWVAFIDSLYDDPSQSANLLAEAKKLNDAQAPK

SEQ ID NO: 511 - protein, 58 aa, artificial sequence
  Modified bacterial sequence
VDAKYAKESIEAWTEIDHLPNLTIEQWLAFINKLTDDPSQSSELLAEAKKLNDAQAPK

SEQ ID NO: 512 - protein, 58 aa, artificial sequence
  Modified bacterial sequence
VDAKYAKEVLDAWHEIDTLPNLTVRQWLAFISKLEDDPSQSSELLAEAKKLNDAQAPK

SEQ ID NO: 513 - protein, 58 aa, artificial sequence
  Modified bacterial sequence
VDAKYAKEHIQANEEIDRLPNLTIKQWLAFINKLHDDPSQSSELLAEAKKLNDAQAPK

SEQ ID NO: 514 - protein, 58 aa, artificial sequence
  Modified bacterial sequence
VDAKYAKEVLHAWAEIDALPNLTIEQWLAFINKLDDDPSQSSELLSEAKKLNDSQAPK

SEQ ID NO: 515 - protein, 58 aa, artificial sequence
  Modified bacterial sequence
VDAKYAKEVLAAWDEIDSLPNLTLQQWLAFINKLDDDPSQSSELLSEAKKLNDSQAPK

SEQ ID NO: 516 - protein, 58 aa, artificial sequence
  Modified bacterial sequence
VDAKYAKEVIDAWNEIDALPNLTLEQWLAFINKLDDDPSQSSELLSEAKKLNDSQAPK

SEQ ID NO: 517 - protein, 58 aa, artificial sequence
  Modified bacterial sequence
VDAKYAKEVLDAWNEIDALPNLTIDQWLAFINKLSDDPSQSSELLSEAKKLNDSQAPK

SEQ ID NO: 518 - protein, 58 aa, artificial sequence
  Modified bacterial sequence
VDAKYAKEVIEAWDEIDGLPNLTIEQWLAFINKLDDDPSQSSELLSEAKKLNDSQAPK

SEQ ID NO: 519 - protein, 58 aa, artificial sequence
  Modified bacterial sequence
VDAKYAKEVLEAWDEIDHLPNLTLQQWLAFINKLDDDPSQSSELLSEAKKLNDSQAPK

SEQ ID NO: 520 - protein, 58 aa, artificial sequence
  Modified bacterial sequence
VDAKYAKEVIEAWNEIDALPNLTIEQWLAFINKLDDDPSQSSELLSEAKKLNDSQAPK

SEQ ID NO: 521 - protein, 58 aa, artificial sequence
  Modified bacterial sequence
VDAKYAKEVIAAWNEIDRLPNLTLTQWLAFINKLDDDPSQSSELLSEAKKLNDSQAPK

SEQ ID NO: 522 - protein, 58 aa, artificial sequence
  Modified bacterial sequence
VDAKYAKEVIEAWDEIDALPNLTLQQWLAFINKLDDDPSQSSELLSEAKKLNDSQAPK

SEQ ID NO: 523 - protein, 58 aa, artificial sequence
  Modified bacterial sequence
VDAKYAKEVIAAWDEIDKLPNLTIEQWLAFINKLDDDPSQSSELLSEAKKLNDSQAPK

SEQ ID NO: 524 - protein, 58 aa, artificial sequence
  Modified bacterial sequence
VDAKYAKEVIAAWDEIDKLPNLTLQQWLAFINKLDDDPSQSSELLSEAKKLNDSQAPK

SEQ ID NO: 525 - protein, 58 aa, artificial sequence
  Modified bacterial sequence
VDAKYAKETIAAWDEIDKLPNLTIEQWLAFINKLDDDPSQSSELLSEAKKLNDSQAPK

SEQ ID NO: 526 - protein, 58 aa, artificial sequence
  Modified bacterial sequence
VDAKYAKETIEAWNEIDRLPNLTIEQWLAFINKLDDDPSQSSELLSEAKKLNDSQAPK

SEQ ID NO: 527 - protein, 58 aa, artificial sequence
  Modified bacterial sequence
VDAKYAKEVLEAWREIDALPNLTIQQWLAFINKLDDDPSQSSELLSEAKKLNDSQAPK

SEQ ID NO: 528 - protein, 58 aa, artificial sequence
  Modified bacterial sequence
VDAKYAKEVIEAWDEIDQLPNLTIEQWLAFINKLDDDPSQSSELLSEAKKLNDSQAPK

SEQ ID NO: 529 - protein, 58 aa, artificial sequence
  Modified bacterial sequence
VDAKYAKEVLRAWDEIDHLPNLTLEQWLAFINKLDDDPSQSSELLSEAKKLNDSQAPK

SEQ ID NO: 530 - protein, 58 aa, artificial sequence
  Modified bacterial sequence
VDAKYAKEVLEAWDEIDRLPNLTLNQWLAFINKLDDDPSQSSELLSEAKKLNDSQAPK

SEQ ID NO: 531 - protein, 58 aa, artificial sequence
  Modified bacterial sequence
VDAKYAKEVLDAWNEIDHLPNLTIEQWLAFINKLDDDPSQSSELLSEAKKLNDSQAPK

SEQ ID NO: 532 - protein, 58 aa, artificial sequence
  Modified bacterial sequence
VDAKYAKEVIDAWNEIDKLPNLTIEQWLAFINKLDDDPSQSSELLSEAKKLNDSQAPK

SEQ ID NO: 533 - protein, 58 aa, artificial sequence
  Modified bacterial sequence
VDAKYAKETLEAWDEIDQLPNLTLQQWLAFINKLDDDPSQSSELLSEAKKLNDSQAPK

SEQ ID NO: 534 - protein, 58 aa, artificial sequence
  Modified bacterial sequence
VDAKYAKEVIEAWNEIDALPNLTLDQWLAFINKLDDDPSQSSELLSEAKKLNDSQAPK

SEQ ID NO: 535 - protein, 58 aa, artificial sequence
  Modified bacterial sequence
VDAKYAKEVIDAWNEIDRLPNLTLQQWLAFINKLDDDPSQSSELLSEAKKLNDSQAPK

SEQ ID NO: 536 - protein, 58 aa, artificial sequence
  Modified bacterial sequence
VDAKYAKEVIDAWNEIDQLPNLTLEQWLAFINKLDDDPSQSSELLSEAKKLNDSQAPK

SEQ ID NO: 537 - protein, 58 aa, artificial sequence
  Modified bacterial sequence
VDAKYAKETIAAWDEIDHLPNLTLEQWLAFINKLDDDPSQSSELLSEAKKLNDSQAPK

SEQ ID NO: 538 - protein, 58 aa, artificial sequence
  Modified bacterial sequence
VDAKYAKEVLQAWDEIDHLPNLTIQQWLAFINKLSDDPSQSSELLSEAKKLNDSQAPK

SEQ ID NO: 539 - protein, 58 aa, artificial sequence
  Modified bacterial sequence
VDAKYAKETLHAWAEIDRLPNLTIEQWLAFINKLDDDPSQSSELLSEAKKLNDSQAPK

SEQ ID NO: 540 - protein, 58 aa, artificial sequence
  Modified bacterial sequence
VDAKYAKEVLEAWNEIDHLPNLTLAQWLAFINKLDDDPSQSSELLSEAKKLNDSQAPK

SEQ ID NO: 541 - protein, 58 aa, artificial sequence
  Modified bacterial sequence
VDAKYAKEVIEAWDEIDKLPNLTIAQWLAFINKLDDDPSQSSELLSEAKKLNDSQAPK

SEQ ID NO: 542 - protein, 58 aa, artificial sequence
  Modified bacterial sequence
VDAKYAKEVLDAWDEIDHLPNLTLQQWLAFINKLDDDPSQSSELLSEAKKLNDSQAPK

SEQ ID NO: 543 - protein, 58 aa, artificial sequence
  Modified bacterial sequence
VDAKYAKETIEAWNEIDKLPNLTLTQWLAFINKLDDDPSQSSELLSEAKKLNDSQAPK

SEQ ID NO: 544 - protein, 58 aa, artificial sequence
  Modified bacterial sequence
VDAKYAKEVLEAWNEIDLLPNLTIEQWLAFINKLDDDPSQSSELLSEAKKLNDSQAPK

SEQ ID NO: 545 - protein, 58 aa, artificial sequence
  Modified bacterial sequence
VDAKYAKEVIEAWDEIDHLPNLTIDQWLAFINKLDDDPSQSSELLSEAKKLNDSQAPK

SEQ ID NO: 546 - protein, 58 aa, artificial sequence
  Modified bacterial sequence
VDAKYAKEVISAWNEIDALPNLTLQQWLAFINKLDDDPSQSSELLSEAKKLNDSQAPK

SEQ ID NO: 547 - protein, 58 aa, artificial sequence
  Modified bacterial sequence
VDAKYAKEVIAAWNEIDKLPNLTLEQWLAFINKLDDDPSQSSELLSEAKKLNDSQAPK

SEQ ID NO: 548 - protein, 58 aa, artificial sequence
  Modified bacterial sequence
VDAKYAKETIEAWNEIDSLPNLTLDQWLAFINKLDDDPSQSSELLSEAKKLNDSQAPK

SEQ ID NO: 549 - protein, 58 aa, artificial sequence
  Modified bacterial sequence
VDAKYAKEVLDAWNEIDQLPNLTLQQWLAFINKLDDDPSQSSELLSEAKKLNDSQAPK

SEQ ID NO: 550 - protein, 58 aa, artificial sequence
  Modified bacterial sequence
VDAKYAKEVLAAWNEIDHLPNLTIEQWLAFINKLDDDPSQSSELLSEAKKLNDSQAPK

SEQ ID NO: 551 - protein, 58 aa, artificial sequence
  Modified bacterial sequence
VDAKYAKEVLEAWDEIDHLPNLTITQWLAFINKLDDDPSQSSELLSEAKKLNDSQAPK

SEQ ID NO: 552 - protein, 58 aa, artificial sequence
  Modified bacterial sequence
VDAKYAKETIDAWNEIDHLPNLTIEQWLAFINKLDDDPSQSSELLSEAKKLNDSQAPK

SEQ ID NO: 553 - protein, 58 aa, artificial sequence
  Modified bacterial sequence
VDAKYAKEVIEAWNEIDHLPNLTIQQWLAFINKLDDDPSQSSELLSEAKKLNDSQAPK

SEQ ID NO: 554 - protein, 58 aa, artificial sequence
  Modified bacterial sequence
VDAKYAKEVIQAWNEIDALPNLTISQWLAFINKLDDDPSQSSELLSEAKKLNDSQAPK

SEQ ID NO: 555 - protein, 58 aa, artificial sequence
  Modified bacterial sequence
VDAKYAKEVIAAWDEIDSLPNLTIEQWLAFINKLDDDPSQSSELLSEAKKLNDSQAPK

SEQ ID NO: 556 - protein, 58 aa, artificial sequence
  Modified bacterial sequence
VDAKYAKEHIEAWNEIDALPNLTIEQWLAFINKLQDDPSQSSELLSEAKKLNDSQAPK

SEQ ID NO: 557 - protein, 58 aa, artificial sequence
  Modified bacterial sequence
VDAKYAKEVLEAWNEIDKLPNLTLDQWLAFINKLDDDPSQSSELLSEAKKLNDSQAPK

SEQ ID NO: 558 - protein, 58 aa, artificial sequence
  Modified bacterial sequence
VDAKYAKEVIDAWNEIDHLPNLTIEQWLAFINKLADDPSQSSELLSEAKKLNDSQAPK

SEQ ID NO: 559 - protein, 58 aa, artificial sequence
  Modified bacterial sequence
VDAKYAKETIDAWDEIDKLPNLTIEQWLAFINKLDDDPSQSSELLSEAKKLNDSQAPK

SEQ ID NO: 560 - protein, 58 aa, artificial sequence
  Modified bacterial sequence
VDAKYAKEVIAAWDEIDLLPNLTLQQWLAFINKLADDPSQSSELLSEAKKLNDSQAPK

SEQ ID NO: 561 - protein, 58 aa, artificial sequence
  Modified bacterial sequence
VDAKYAKEVIHAWDEIDKLPNLTIEQWLAFINKLDDDPSQSSELLSEAKKLNDSQAPK

SEQ ID NO: 562 - protein, 58 aa, artificial sequence
  Modified bacterial sequence
VDAKYAKEVIAAWNEIDHLPNLTLEQWLAFINKLDDDPSQSSELLSEAKKLNDSQAPK

SEQ ID NO: 563 - protein, 58 aa, artificial sequence
  Modified bacterial sequence
VDAKYAKETLDAWNEIDKLPNLTLSQWLAFINKLDDDPSQSSELLSEAKKLNDSQAPK

SEQ ID NO: 564 - protein, 58 aa, artificial sequence
  Modified bacterial sequence
VDAKYAKEVLEAWNEIDALPNLTLEQWLAFINKLDDDPSQSSELLSEAKKLNDSQAPK

SEQ ID NO: 565 - protein, 58 aa, artificial sequence
  Modified bacterial sequence
VDAKYAKEVIQAWDEIDHLPNLTISQWLAFINKLDDDPSQSSELLSEAKKLNDSQAPK

SEQ ID NO: 566 - protein, 58 aa, artificial sequence
  Modified bacterial sequence
VDAKYAKEVLQAWDEIDSLPNLTIEQWLAFINKLDDDPSQSSELLSEAKKLNDSQAPK

SEQ ID NO: 567 - protein, 58 aa, artificial sequence
  Modified bacterial sequence
VDAKYAKETLEAWDEIDHLPNLTIAQWLAFINKLDDDPSQSSELLSEAKKLNDSQAPK

SEQ ID NO: 568 - protein, 58 aa, artificial sequence
  Modified bacterial sequence
VDAKYAKETIDAWNEIDRLPNLTISQWLAFINKLDDDPSQSSELLSEAKKLNDSQAPK

SEQ ID NO: 569 - protein, 58 aa, artificial sequence
  Modified bacterial sequence
VDAKYAKEVLDAWHEIDHLPNLTIQQWLAFINKLDDDPSQSSELLSEAKKLNDSQAPK

SEQ ID NO: 570 - protein, 58 aa, artificial sequence
  Modified bacterial sequence
VDAKYAKEQIRAWDEIDKLPNLTIEQWLAFINKLADDPSQSSELLSEAKKLNDSQAPK

SEQ ID NO: 571 - protein, 58 aa, artificial sequence
  Modified bacterial sequence
VDAKYAKETLYAWNEIDKLPNLTIEQWLAFIEKLQDDPSQSSELLSEAKKLNDSQAPK

SEQ ID NO: 572 - protein, 58 aa, artificial sequence
  Modified bacterial sequence
VDAKYAKEVIEAWNEIDALPNLTIDQWLAFINKLDDDPSQSSELLSEAKKLNDSQAPK

SEQ ID NO: 573 - protein, 58 aa, artificial sequence
  Modified bacterial sequence
VDAKYAKEVLEAWNEIDHLPNLTIQQWLAFINKLDDDPSQSSELLSEAKKLNDSQAPK

SEQ ID NO: 574 - protein, 58 aa, artificial sequence
  Modified bacterial sequence
VDAKYAKETIEAWDEIDALPNLTIEQWLAFINKLDDDPSQSSELLSEAKKLNDSQAPK

SEQ ID NO: 575 - protein, 58 aa, artificial sequence
  Modified bacterial sequence
VDAKYAKEVIEAWNEIDHLPNLTLQQWLAFINKLDDDPSQSSELLSEAKKLNDSQAPK

SEQ ID NO: 576 - protein, 58 aa, artificial sequence
  Modified bacterial sequence
VDAKYAKEVIEAWNEIDKLPNLTIQQWLAFINKLDDDPSQSSELLSEAKKLNDSQAPK

SEQ ID NO: 577 - protein, 58 aa, artificial sequence
  Modified bacterial sequence
VDAKYAKETLDAWAEIDHLPNLTLDQWLAFINKLDDDPSQSSELLSEAKKLNDSQAPK

SEQ ID NO: 578 - protein, 58 aa, artificial sequence
  Modified bacterial sequence
VDAKYAKEHIDAWNEIDALPNLTLSQWLAFINKLDDDPSQSSELLSEAKKLNDSQAPK

SEQ ID NO: 579 - protein, 58 aa, artificial sequence
  Modified bacterial sequence
VDAKYAKEVLDAWNEIDKLPNLTIAQWLAFINKLDDDPSQSSELLSEAKKLNDSQAPK

SEQ ID NO: 580 - protein, 58 aa, artificial sequence
  Modified bacterial sequence
VDAKYAKEVIEAWTEIDYLPNLTLQQWLAFINKLDDDPSQSSELLSEAKKLNDSQAPK

SEQ ID NO: 581 - protein, 58 aa, artificial sequence
  Modified bacterial sequence
VDAKYAKETIEAWNEIDHLPNLTIAQWLAFINKLDDDPSQSSELLSEAKKLNDSQAPK

SEQ ID NO: 582 - protein, 58 aa, artificial sequence
  Modified bacterial sequence
VDAKYAKEVIQAWNEIDKLPNLTLEQWLAFINKLDDDPSQSSELLSEAKKLNDSQAPK

SEQ ID NO: 583 - protein, 58 aa, artificial sequence
  Modified bacterial sequence
VDAKYAKEVIEAWDEIDHLPNLTIEQWLAFINKLDDDPSQSSELLSEAKKLNDSQAPK

SEQ ID NO: 584 - protein, 58 aa, artificial sequence
  Modified bacterial sequence
VDAKYAKETIDAWNEIDLLPNLTIEQWLAFINKLDDDPSQSSELLSEAKKLNDSQAPK

SEQ ID NO: 585 - protein, 58 aa, artificial sequence
  Modified bacterial sequence
VDAKYAKEHIDAWNEIDKLPNLTLDQWLAFINKLDDDPSQSSELLSEAKKLNDSQAPK

SEQ ID NO: 586 - protein, 58 aa, artificial sequence
  Modified bacterial sequence
VDAKYAKEVVAAWNEIDALPNLTIEQWLAFINKLNDDPSQSSELLSEAKKLNDSQAPK

SEQ ID NO: 587 - protein, 58 aa, artificial sequence
  Modified bacterial sequence
VDAKYAKEVIEAWNEIDALPNLTLAQWLAFINKLDDDPSQSSELLSEAKKLNDSQAPK

SEQ ID NO: 588 - protein, 58 aa, artificial sequence
  Modified bacterial sequence
VDAKYAKEVLQAWDEIDRLPNLTLDQWLAFINKLDDDPSQSSELLSEAKKLNDSQAPK

SEQ ID NO: 589 - protein, 58 aa, artificial sequence
  Modified bacterial sequence
VDAKYAKEVIDAWDEIDHLPNLTIEQWLAFINKLSDDPSQSSELLSEAKKLNDSQAPK

SEQ ID NO: 590 - protein, 58 aa, artificial sequence
  Modified bacterial sequence
VDAKYAKEVVEAWNEIDQLPNLTIEQWLAFINKLDDDPSQSSELLSEAKKLNDSQAPK

SEQ ID NO: 591 - protein, 58 aa, artificial sequence
  Modified bacterial sequence
VDAKYAKEVIQAWNEIDALPNLTIEQWLAFINKLDDDPSQSSELLSEAKKLNDSQAPK

SEQ ID NO: 592 - protein, 58 aa, artificial sequence
  Modified bacterial sequence
VDAKYAKEVIQAWDEIDKLPNLTIDQWLAFINKLADDPSQSSELLSEAKKLNDSQAPK

SEQ ID NO: 593 - protein, 58 aa, artificial sequence
  Modified bacterial sequence
VDAKYAKEVVAAWDEIDALPNLTLTQWLAFINKLDDDPSQSSELLSEAKKLNDSQAPK

SEQ ID NO: 594 - protein, 58 aa, artificial sequence
  Modified bacterial sequence
VDAKYAKEVIQAWNEIDGLPNLTLSQWLAFINKLDDDPSQSSELLSEAKKLNDSQAPK

SEQ ID NO: 595 - protein, 58 aa, artificial sequence
  Modified bacterial sequence
VDAKYAKETIEAWDEIDALPNLTITQWLAFINKLDDDPSQSSELLSEAKKLNDSQAPK

SEQ ID NO: 596 - protein, 58 aa, artificial sequence
  Modified bacterial sequence
VDAKYAKEVIDAWNEIDHLPNLTIQQWLAFINKLADDPSQSSELLSEAKKLNDSQAPK

SEQ ID NO: 597 - protein, 58 aa, artificial sequence
  Modified bacterial sequence
VDAKYAKETIEAWNEIDALPNLTLDQWLAFINKLEDDPSQSSELLSEAKKLNDSQAPK

SEQ ID NO: 598 - protein, 58 aa, artificial sequence
  Modified bacterial sequence
VDAKYAKEHIHAWNEIDELPNLTIEQWLAFINKLADDPSQSSELLSEAKKLNDSQAPK

SEQ ID NO: 599 - protein, 58 aa, artificial sequence
  Modified bacterial sequence
VDAKYAKEVIDAWDEIDHLPNLTIDQWLAFINKLSDDPSQSSELLSEAKKLNDSQAPK

SEQ ID NO: 600 - protein, 58 aa, artificial sequence
  Modified bacterial sequence
VDAKYAKEVIDANDEIDALPNLTIAQWLAFINKLHDDPSQSSELLSEAKKLNDSQAPK

SEQ ID NO: 601 - protein, 58 aa, artificial sequence
  Modified bacterial sequence
VDAKYAKETIEAWDEIDKLPNLTIEQWLAFINKLDDDPSQSSELLSEAKKLNDSQAPK

SEQ ID NO: 602 - protein, 58 aa, artificial sequence
  Modified bacterial sequence
VDAKYAKEVLLAWDEIDHLPNLTLEQWLAFINKLDDDPSQSSELLSEAKKLNDSQAPK

SEQ ID NO: 603 - protein, 58 aa, artificial sequence
  Modified bacterial sequence
VDAKYAKEHIDAWNEIDGLPNLTLEQWLAFINKLDDDPSQSSELLSEAKKLNDSQAPK

SEQ ID NO: 604 - protein, 58 aa, artificial sequence
  Modified bacterial sequence
VDAKYAKEVIEAWSEIDALPNLTIDQWLAFINKLADDPSQSSELLSEAKKLNDSQAPK

SEQ ID NO: 605 - protein, 58 aa, artificial sequence
  Modified bacterial sequence
VDAKYAKEQLNAWAEIDALPNLTIEQWLAFINKLDDDPSQSSELLSEAKKLNDSQAPK

SEQ ID NO: 606 - protein, 58 aa, artificial sequence
  Modified bacterial sequence
VDAKYAKEVIDAWNEIDALPNLTIAQWLAFINKLDDDPSQSSELLSEAKKLNDSQAPK

SEQ ID NO: 607 - protein, 58 aa, artificial sequence
  Modified bacterial sequence
VDAKYAKETIDAWNEIDQLPNLTIEQWLAFINKLDDDPSQSSELLSEAKKLNDSQAPK

SEQ ID NO: 608 - protein, 58 aa, artificial sequence
  Modified bacterial sequence
VDAKYAKEVIEAWDEIDKLPNLTLAQWLAFINKLDDDPSQSSELLSEAKKLNDSQAPK

SEQ ID NO: 609 - protein, 58 aa, artificial sequence
  Modified bacterial sequence
VDAKYAKEVLYAWAEIDHLPNLTIEQWLAFINKLDDDPSQSSELLSEAKKLNDSQAPK

SEQ ID NO: 610 - protein, 58 aa, artificial sequence
  Modified bacterial sequence
VDAKYAKEQIDAWNEIDRLPNLTIQQWLAFINKLDDDPSQSSELLSEAKKLNDSQAPK

SEQ ID NO: 611 - protein, 58 aa, artificial sequence
  Modified bacterial sequence
VDAKYAKEVLAAWDEIDRLPNLTIEQWLAFINKLDDDPSQSSELLSEAKKLNDSQAPK

SEQ ID NO: 612 - protein, 58 aa, artificial sequence
  Modified bacterial sequence
VDAKYAKEVIEAWDEIDHLPNLTLHQWLAFINKLDDDPSQSSELLSEAKKLNDSQAPK

SEQ ID NO: 613 - protein, 58 aa, artificial sequence
  Modified bacterial sequence
VDAKYAKEVIEAWNEIDKLPNLTLQQWLAFINKLDDDPSQSSELLSEAKKLNDSQAPK

SEQ ID NO: 614 - protein, 58 aa, artificial sequence
  Modified bacterial sequence
VDAKYAKEVIDANDEIDALPNLTIEQWLAFINKLHDDPSQSSELLSEAKKLNDSQAPK

SEQ ID NO: 615 - protein, 58 aa, artificial sequence
  Modified bacterial sequence
VDAKYAKEVIAAWDEIDALPNLTIEQWLAFINKLDDDPSQSSELLSEAKKLNDSQAPK

SEQ ID NO: 616 - protein, 58 aa, artificial sequence
  Modified bacterial sequence
VDAKYAKEVIEAWTEIDQLPNLTLDQWLAFINKLDDDPSQSSELLSEAKKLNDSQAPK

SEQ ID NO: 617 - protein, 58 aa, artificial sequence
  Modified bacterial sequence
VDAKYAKEVINAWNEIDALPNLTLQQWLAFINKLDDDPSQSSELLSEAKKLNDSQAPK

SEQ ID NO: 618 - protein, 58 aa, artificial sequence
  Modified bacterial sequence
VDAKYAKEHIEAWDEIDHLPNLTIDQWLAFINKLADDPSQSSELLSEAKKLNDSQAPK

SEQ ID NO: 619 - protein, 58 aa, artificial sequence
  Modified bacterial sequence
VDAKYAKEHLEAWREIDALPNLTIEQWLAFINKLDDDPSQSSELLSEAKKLNDSQAPK

SEQ ID NO: 620 - protein, 58 aa, artificial sequence
  Modified bacterial sequence
VDAKYAKEVLDAWNEIDKLPNLTLQQWLAFINKLDDDPSQSSELLSEAKKLNDSQAPK

SEQ ID NO: 621 - protein, 58 aa, artificial sequence
  Modified bacterial sequence
VDAKYAKEVIAAWDEIDHLPNLTIQQWLAFINKLDDDPSQSSELLSEAKKLNDSQAPK

SEQ ID NO: 622 - protein, 58 aa, artificial sequence
  Modified bacterial sequence
VDAKYAKEVIQAWNEIDALPNLTLEQWLAFINKLDDDPSQSSELLSEAKKLNDSQAPK

SEQ ID NO: 623 - protein, 58 aa, artificial sequence
  Modified bacterial sequence
VDAKYAKEVIDAWNEIDHLPNLTIAQWLAFINKLDDDPSQSSELLSEAKKLNDSQAPK

SEQ ID NO: 624 - protein, 58 aa, artificial sequence
  Modified bacterial sequence
VDAKYAKEQLDAWDEIDHLPNLTIDQWLAFINKLSDDPSQSSELLSEAKKLNDSQAPK

SEQ ID NO: 625 - protein, 58 aa, artificial sequence
  Modified bacterial sequence
VDAKYAKEVLNAWDEIDKLPNLTIEQWLAFINKLDDDPSQSSELLSEAKKLNDSQAPK

SEQ ID NO: 626 - protein, 58 aa, artificial sequence
  Modified bacterial sequence
VDAKYAKEVLEAWNEIDHLPNLTIDQWLAFINKLDDDPSQSSELLSEAKKLNDSQAPK

SEQ ID NO: 627 - protein, 58 aa, artificial sequence
  Modified bacterial sequence
VDAKYAKEVLLAWDEIDRLPNLTIDQWLAFINKLADDPSQSSELLSEAKKLNDSQAPK

SEQ ID NO: 628 - protein, 58 aa, artificial sequence
  Modified bacterial sequence
VDAKYAKEVIAAWNEIDQLPNLTLDQWLAFINKLDDDPSQSSELLSEAKKLNDSQAPK

SEQ ID NO: 629 - protein, 58 aa, artificial sequence
  Modified bacterial sequence
VDAKYAKETLLAWDEIDALPNLTIEQWLAFINKLDDDPSQSSELLSEAKKLNDSQAPK

SEQ ID NO: 630 - protein, 58 aa, artificial sequence
  Modified bacterial sequence
VDAKYAKEVIDAWNEIDTLPNLTLEQWLAFINKLDDDPSQSSELLSEAKKLNDSQAPK

SEQ ID NO: 631 - protein, 58 aa, artificial sequence
  Modified bacterial sequence
VDAKYAKEVLHAWNEIDHLPNLTLNQWLAFINKLQDDPSQSSELLSEAKKLNDSQAPK

SEQ ID NO: 632 - protein, 58 aa, artificial sequence
  Modified bacterial sequence
VDAKYAKEVIQAWNEIDALPNLTIAQWLAFINKLDDDPSQSSELLSEAKKLNDSQAPK

SEQ ID NO: 633 - protein, 58 aa, artificial sequence
  Modified bacterial sequence
VDAKYAKETVDAWNEIDALPNLTIEQWLAFINKLDDDPSQSSELLSEAKKLNDSQAPK

SEQ ID NO: 634 - protein, 58 aa, artificial sequence
  Modified bacterial sequence
VDAKYAKEVIQAWDEIDHLPNLTIDQWLAFINKLDDDPSQSSELLSEAKKLNDSQAPK

SEQ ID NO: 635 - protein, 58 aa, artificial sequence
  Modified bacterial sequence
VDAKYAKEVLDAWNEIDQLPNLTIQQWLAFINKLDDDPSQSSELLSEAKKLNDSQAPK

SEQ ID NO: 636 - protein, 58 aa, artificial sequence
  Modified bacterial sequence
VDAKYAKETIEAWNEIDALPNLTLDQWLAFINKLDDDPSQSSELLSEAKKLNDSQAPK

SEQ ID NO: 637 - protein, 58 aa, artificial sequence
  Modified bacterial sequence
VDAKYAKEVIEAWDEIDALPNLTIDQWLAFINKLDDDPSQSSELLSEAKKLNDSQAPK

SEQ ID NO: 638 - protein, 58 aa, artificial sequence
  Modified bacterial sequence
VDAKYAKEVIEAWNEIDQLPNLTIQQWLAFINKLDDDPSQSSELLSEAKKLNDSQAPK

SEQ ID NO: 639 - protein, 58 aa, artificial sequence
  Modified bacterial sequence
VDAKYAKEVIEAWTEIDHLPNLTIEQWLAFINKLDDDPSQSSELLSEAKKLNDSQAPK

SEQ ID NO: 640 - protein, 58 aa, artificial sequence
  Modified bacterial sequence
VDAKYAKEVIQAWNEIDHLPNLTLQQWLAFINKLEDDPSQSSELLSEAKKLNDSQAPK

SEQ ID NO: 641 - protein, 58 aa, artificial sequence
  Modified bacterial sequence
VDAKYAKEVIQANNEIDQLPNLTIEQWLAFINKLHDDPSQSSELLSEAKKLNDSQAPK

SEQ ID NO: 642 - protein, 58 aa, artificial sequence
  Modified bacterial sequence
VDAKYAKEVLHAWSEIDKLPNLTIEQWLAFINKLDDDPSQSSELLSEAKKLNDSQAPK

SEQ ID NO: 643 - protein, 58 aa, artificial sequence
  Modified bacterial sequence
VDAKYAKETIQAWDEIDKLPNLTLDQWLAFINKLSDDPSQSSELLSEAKKLNDSQAPK

SEQ ID NO: 644 - protein, 58 aa, artificial sequence
  Modified bacterial sequence
VDAKYAKETLRAWDEIDKLPNLTIQQWLAFINKLADDPSQSSELLSEAKKLNDSQAPK

SEQ ID NO: 645 - protein, 58 aa, artificial sequence
  Modified bacterial sequence
VDAKYAKEVIDAWNEIDHLPNLTIEQWLAFINKLEDDPSQSSELLSEAKKLNDSQAPK

SEQ ID NO: 646 - protein, 58 aa, artificial sequence
  Modified bacterial sequence
VDAKYAKEVIDAWNEIDHLPNLTLQQWLAFINKLADDPSQSSELLSEAKKLNDSQAPK

SEQ ID NO: 647 - protein, 58 aa, artificial sequence
  Modified bacterial sequence
VDAKYAKETIDAWNEIDALPNLTLDQWLAFINKLDDDPSQSSELLSEAKKLNDSQAPK

SEQ ID NO: 648 - protein, 58 aa, artificial sequence
  Modified bacterial sequence
VDAKYAKEVIEAWNEIDQLPNLTIEQWLAFINKLDDDPSQSSELLSEAKKLNDSQAPK

SEQ ID NO: 649 - protein, 58 aa, artificial sequence
  Modified bacterial sequence
VDAKYAKEVIRAWDEIDQLPNLTLSQWLAFINKLDDDPSQSSELLSEAKKLNDSQAPK

SEQ ID NO: 650 - protein, 58 aa, artificial sequence
  Modified bacterial sequence
VDAKYAKEVIEAWNEIDRLPNLTIHQWLAFINKLDDDPSQSSELLSEAKKLNDSQAPK

SEQ ID NO: 651 - protein, 58 aa, artificial sequence
  Modified bacterial sequence
VDAKYAKETIEAWNEIDQLPNLTIEQWLAFINKLDDDPSQSSELLSEAKKLNDSQAPK

SEQ ID NO: 652 - protein, 58 aa, artificial sequence
  Modified bacterial sequence
VDAKYAKEVLTAWAEIDALPNLTLSQWLAFINKLDDDPSQSSELLSEAKKLNDSQAPK

SEQ ID NO: 653 - protein, 58 aa, artificial sequence
  Modified bacterial sequence
VDAKYAKEVIEAWDEIDKLPNLTVDQWLAFINKLDDDPSQSSELLSEAKKLNDSQAPK

SEQ ID NO: 654 - protein, 58 aa, artificial sequence
  Modified bacterial sequence
VDAKYAKEVIDAWNEIDHLPNLTLTQWLAFINKLDDDPSQSSELLSEAKKLNDSQAPK

SEQ ID NO: 655 - protein, 58 aa, artificial sequence
  Modified bacterial sequence
VDAKYAKEVIEAWNEIDQLPNLTLDQWLAFINKLDDDPSQSSELLSEAKKLNDSQAPK

SEQ ID NO: 656 - protein, 58 aa, artificial sequence
  Modified bacterial sequence
VDAKYAKETLQAWDEIDHLPNLTLNQWLAFINKLDDDPSQSSELLSEAKKLNDSQAPK

SEQ ID NO: 657 - protein, 58 aa, artificial sequence
  Modified bacterial sequence
VDAKYAKEVIDAWNEIDHLPNLTIEQWLAFINKLDDDPSQSSELLSEAKKLNDSQAPK

SEQ ID NO: 658 - protein, 58 aa, artificial sequence
  Modified bacterial sequence
VDAKYAKEVIEAWNEIDLLPNLTLSQWLAFINKLDDDPSQSSELLSEAKKLNDSQAPK

SEQ ID NO: 659 - protein, 58 aa, artificial sequence
  Modified bacterial sequence
VDAKYAKEVIDAWDEIDRLPNLTLKQWLAFINKLDDDPSQSSELLSEAKKLNDSQAPK

SEQ ID NO: 660 - protein, 58 aa, artificial sequence
  Modified bacterial sequence
VDAKYAKETLHAWDEIDKLPNLTIEQWLAFINKLDDDPSQSSELLSEAKKLNDSQAPK

SEQ ID NO: 661 - protein, 58 aa, artificial sequence
  Modified bacterial sequence
VDAKYAKEVIKAWDEIDHLPNLTLNQWLAFINKLDDDPSQSSELLSEAKKLNDSQAPK

SEQ ID NO: 662 - protein, 58 aa, artificial sequence
  Modified bacterial sequence
VDAKYAKEVIEAWNEIDHLPNLTLAQWLAFINKLDDDPSQSSELLSEAKKLNDSQAPK

SEQ ID NO: 663 - protein, 58 aa, artificial sequence
  Modified bacterial sequence
VDAKYAKEVIQAWNEIDHLPNLTIDQWLAFITKLEDDPSQSSELLSEAKKLNDSQAPK

SEQ ID NO: 664 - protein, 58 aa, artificial sequence
  Modified bacterial sequence
VDAKYAKEVIEAWNEIDRLPNLTIKQWLAFINKLDDDPSQSSELLSEAKKLNDSQAPK

SEQ ID NO: 665 - protein, 58 aa, artificial sequence
  Modified bacterial sequence
VDAKYAKEVIEAWNEIDSLPNLTLQQWLAFINKLDDDPSQSSELLSEAKKLNDSQAPK

SEQ ID NO: 666 - protein, 58 aa, artificial sequence
  Modified bacterial sequence
VDAKYAKETIDAWNEIDKLPNLTIEQWLAFINKLDDDPSQSSELLSEAKKLNDSQAPK

SEQ ID NO: 667 - protein, 58 aa, artificial sequence
  Modified bacterial sequence
VDAKYAKEVLEAWAEIDALPNLTIAQWLAFINKLDDDPSQSSELLSEAKKLNDSQAPK

SEQ ID NO: 668 - protein, 58 aa, artificial sequence
  Modified bacterial sequence
VDAKYAKETIDAWNEIDRLPNLTIEQWLAFINKLDDDPSQSSELLSEAKKLNDSQAPK

SEQ ID NO: 669 - protein, 58 aa, artificial sequence
  Modified bacterial sequence
VDAKYAKETLKAWDEIDRLPNLTLEQWLAFINKLDDDPSQSSELLSEAKKLNDSQAPK

SEQ ID NO: 670 - protein, 58 aa, artificial sequence
  Modified bacterial sequence
VDAKYAKETIAAWNEIDALPNLTLQQWLAFINKLDDDPSQSSELLSEAKKLNDSQAPK

SEQ ID NO: 671 - protein, 58 aa, artificial sequence
  Modified bacterial sequence
VDAKYAKEVLQAWNEIDHLPNLTIQQWLAFINKLDDDPSQSSELLSEAKKLNDSQAPK

SEQ ID NO: 672 - protein, 58 aa, artificial sequence
  Modified bacterial sequence
VDAKYAKEVIEAWSEIDHLPNLTLQQWLAFINKLDDDPSQSSELLSEAKKLNDSQAPK

SEQ ID NO: 673 - protein, 58 aa, artificial sequence
  Modified bacterial sequence
VDAKYAKEVIDAWNEIDGLPNLTIEQWLAFINKLDDDPSQSSELLSEAKKLNDSQAPK

SEQ ID NO: 674 - protein, 58 aa, artificial sequence
  Modified bacterial sequence
VDAKYAKEVIHAWNEIDHLPNLTLNQWLAFINKLEDDPSQSSELLSEAKKLNDSQAPK

SEQ ID NO: 675 - protein, 58 aa, artificial sequence
  Modified bacterial sequence
VDAKYAKEVLDAWNEIDSLPNLTLDQWLAFINKLDDDPSQSSELLSEAKKLNDSQAPK

SEQ ID NO: 676 - protein, 58 aa, artificial sequence
  Modified bacterial sequence
VDAKYAKEQIEAWNEIDRLPNLTLEQWLAFINKLDDDPSQSSELLSEAKKLNDSQAPK

SEQ ID NO: 677 - protein, 58 aa, artificial sequence
  Modified bacterial sequence
VDAKYAKEVVDAWNEIDALPNLTLQQWLAFINKLDDDPSQSSELLSEAKKLNDSQAPK

SEQ ID NO: 678 - protein, 58 aa, artificial sequence
  Modified bacterial sequence
VDAKYAKEVIEAWNEIDKLPNLTIEQWLAFINKLDDDPSQSSELLSEAKKLNDSQAPK

SEQ ID NO: 679 - protein, 58 aa, artificial sequence
  Modified bacterial sequence
VDAKYAKEVIEANDEIDRLPNLTIEQWLAFINKLHDDPSQSSELLSEAKKLNDSQAPK

SEQ ID NO: 680 - protein, 58 aa, artificial sequence
  Modified bacterial sequence
VDAKYAKETLQAWDEIDKLPNLTIEQWLAFINKLDDDPSQSSELLSEAKKLNDSQAPK

SEQ ID NO: 681 - protein, 58 aa, artificial sequence
  Modified bacterial sequence
VDAKYAKEVIEAWDEIDHLPNLTIDQWLAFINKLADDPSQSSELLSEAKKLNDSQAPK

SEQ ID NO: 682 - protein, 58 aa, artificial sequence
  Modified bacterial sequence
VDAKYAKETIDAWNEIDHLPNLTLQQWLAFINKLADDPSQSSELLSEAKKLNDSQAPK

SEQ ID NO: 683 - protein, 58 aa, artificial sequence
  Modified bacterial sequence
VDAKYAKEVIDAWDEIDKLPNLTIEQWLAFINKLDDDPSQSSELLSEAKKLNDSQAPK

SEQ ID NO: 684 - protein, 58 aa, artificial sequence
  Modified bacterial sequence
VDAKYAKEVIEAWNEIDKLPNLTLAQWLAFINKLDDDPSQSSELLSEAKKLNDSQAPK

SEQ ID NO: 685 - protein, 58 aa, artificial sequence
  Modified bacterial sequence
VDAKYAKEVLQAWDEIDKLPNLTIQQWLAFINKLDDDPSQSSELLSEAKKLNDSQAPK

SEQ ID NO: 686 - protein, 58 aa, artificial sequence
  Modified bacterial sequence
VDAKYAKEVIAAWNEIDGLPNLTLQQWLAFINKLDDDPSQSSELLSEAKKLNDSQAPK

SEQ ID NO: 687 - protein, 58 aa, artificial sequence
  Modified bacterial sequence
VDAKYAKETLNAWNEIDALPNLTLQQWLAFINKLDDDPSQSSELLSEAKKLNDSQAPK

SEQ ID NO: 688 - protein, 58 aa, artificial sequence
  Modified bacterial sequence
VDAKYAKEVLSAWNEIDQLPNLTLEQWLAFINKLDDDPSQSSELLSEAKKLNDSQAPK

SEQ ID NO: 689 - protein, 58 aa, artificial sequence
  Modified bacterial sequence
VDAKYAKETLEAWDEIDHLPNLTLHQWLAFINKLDDDPSQSSELLSEAKKLNDSQAPK

SEQ ID NO: 690 - protein, 58 aa, artificial sequence
  Modified bacterial sequence
VDAKYAKEQIEAWNEIDHLPNLTLQQWLAFINKLADDPSQSSELLSEAKKLNDSQAPK

SEQ ID NO: 691 - protein, 58 aa, artificial sequence
  Modified bacterial sequence
VDAKYAKEVVEAWDEIDKLPNLTIEQWLAFINKLDDDPSQSSELLSEAKKLNDSQAPK

SEQ ID NO: 692 - protein, 58 aa, artificial sequence
  Modified bacterial sequence
VDAKYAKEVLEAWNEIDELPNLTIEQWLAFINKLDDDPSQSSELLSEAKKLNDSQAPK

SEQ ID NO: 693 - protein, 58 aa, artificial sequence
  Modified bacterial sequence
VDAKYAKEVIDAWNEIDQLPNLTLQQWLAFINKLDDDPSQSSELLSEAKKLNDSQAPK

SEQ ID NO: 694 - protein, 58 aa, artificial sequence
  Modified bacterial sequence
VDAKYAKETIDAWDEIDKLPNLTLSQWLAFINKLDDDPSQSSELLSEAKKLNDSQAPK

SEQ ID NO: 695 - protein, 58 aa, artificial sequence
  Modified bacterial sequence
VDAKYAKETIDAWNEIDQLPNLTLQQWLAFINKLDDDPSQSSELLSEAKKLNDSQAPK

SEQ ID NO: 696 - protein, 58 aa, artificial sequence
  Modified bacterial sequence
VDAKYAKEVIQAWDEIDALPNLTLNQWLAFINKLDDDPSQSSELLSEAKKLNDSQAPK

SEQ ID NO: 697 - protein, 58 aa, artificial sequence
  Modified bacterial sequence
VDAKYAKEVLDAWAEIDQLPNLTLQQWLAFINKLDDDPSQSSELLSEAKKLNDSQAPK

SEQ ID NO: 698 - protein, 58 aa, artificial sequence
  Modified bacterial sequence
VDAKYAKEHIAAWDEIDALPNLTIEQWLAFINKLDDDPSQSSELLSEAKKLNDSQAPK

SEQ ID NO: 699 - protein, 58 aa, artificial sequence
  Modified bacterial sequence
VDAKYAKEVIRAWDEIDALPNLTIEQWLAFINKLDDDPSQSSELLSEAKKLNDSQAPK

SEQ ID NO: 700 - protein, 58 aa, artificial sequence
  Modified bacterial sequence
VDAKYAKEVIDAWDEIDALPNLTIDQWLAFINKLADDPSQSSELLSEAKKLNDSQAPK

SEQ ID NO: 701 - protein, 58 aa, artificial sequence
  Modified bacterial sequence
VDAKYAKEVIDAWNEIDRLPNLTIQQWLAFINKLDDDPSQSSELLSEAKKLNDSQAPK

SEQ ID NO: 702 - protein, 58 aa, artificial sequence
  Modified bacterial sequence
VDAKYAKEVITAWNEIDHLPNLTLSQWLAFINKLDDDPSQSSELLSEAKKLNDSQAPK

SEQ ID NO: 703 - protein, 58 aa, artificial sequence
  Modified bacterial sequence
VDAKYAKEVIDAWNEIDALPNLTIHQWLAFINKLDDDPSQSSELLSEAKKLNDSQAPK

SEQ ID NO: 704 - protein, 58 aa, artificial sequence
  Modified bacterial sequence
VDAKYAKEQLKAWDEIDKLPNLTIEQWLAFIEKLQDDPSQSSELLSEAKKLNDSQAPK

SEQ ID NO: 705 - protein, 58 aa, artificial sequence
  Modified bacterial sequence
VDAKYAKEHIDAWTEIDHLPNLTIEQWLAFINKLDDDPSQSSELLSEAKKLNDSQAPK

SEQ ID NO: 706 - protein, 58 aa, artificial sequence
  Modified bacterial sequence
VDAKYAKEQLRAWDEIDKLPNLTIEQWLAFINKLQDDPSQSSELLSEAKKLNDSQAPK

SEQ ID NO: 707 - protein, 58 aa, artificial sequence
  Modified bacterial sequence
VDAKYAKEVLEAWREIDSLPNLTIAQWLAFINKLDDDPSQSSELLSEAKKLNDSQAPK

SEQ ID NO: 708 - protein, 58 aa, artificial sequence
  Modified bacterial sequence
VDAKYAKEVIQAWNEIDKLPNLTIEQWLAFINKLDDDPSQSSELLSEAKKLNDSQAPK

SEQ ID NO: 709 - protein, 58 aa, artificial sequence
  Modified bacterial sequence
VDAKYAKEHVEAWNEIDQLPNLTIEQWLAFINKLADDPSQSSELLSEAKKLNDSQAPK

SEQ ID NO: 710 - protein, 58 aa, artificial sequence
  Modified bacterial sequence
VDAKYAKEVIDAWDEIDALPNLTIDQWLAFINKLSDDPSQSSELLSEAKKLNDSQAPK

SEQ ID NO: 711 - protein, 58 aa, artificial sequence
  Modified bacterial sequence
VDAKYAKEVIEAWNEIDHLPNLTIEQWLAFINKLDDDPSQSSELLSEAKKLNDSQAPK

SEQ ID NO: 712 - protein, 58 aa, artificial sequence
  Modified bacterial sequence
VDAKYAKEVLQAWDEIDKLPNLTIEQWLAFINKLSDDPSQSSELLSEAKKLNDSQAPK

SEQ ID NO: 713 - protein, 58 aa, artificial sequence
  Modified bacterial sequence
VDAKYAKEVIKAWNEIDSLPNLTIEQWLAFINKLDDDPSQSSELLSEAKKLNDSQAPK

SEQ ID NO: 714 - protein, 58 aa, artificial sequence
  Modified bacterial sequence
VDAKYAKEVLEAWHEIDLLPNLTIQQWLAFINKLDDDPSQSSELLSEAKKLNDSQAPK

SEQ ID NO: 715 - protein, 58 aa, artificial sequence
  Modified bacterial sequence
VDAKYAKEVLEAWTEIDRLPNLTLDQWLAFINKLDDDPSQSSELLSEAKKLNDSQAPK

SEQ ID NO: 716 - protein, 58 aa, artificial sequence
  Modified bacterial sequence
VDAKYAKEQLYAWNEIDHLPNLTIEQWLAFIEKLQDDPSQSSELLSEAKKLNDSQAPK

SEQ ID NO: 717 - protein, 58 aa, artificial sequence
  Modified bacterial sequence
VDAKYAKEVLNAWDEIDKLPNLTIKQWLAFINKLDDDPSQSSELLSEAKKLNDSQAPK

SEQ ID NO: 718 - protein, 58 aa, artificial sequence
  Modified bacterial sequence
VDAKYAKEVIRAWDEIDKLPNLTVEQWLAFINKLDDDPSQSSELLSEAKKLNDSQAPK

SEQ ID NO: 719 - protein, 58 aa, artificial sequence
  Modified bacterial sequence
VDAKYAKEVVQAWDEIDQLPNLTLEQWLAFINKLDDDPSQSSELLSEAKKLNDSQAPK

SEQ ID NO: 720 - protein, 58 aa, artificial sequence
  Modified bacterial sequence
VDAKYAKEVIRAWDEIDQLPNLTLEQWLAFINKLDDDPSQSSELLSEAKKLNDSQAPK

SEQ ID NO: 721 - protein, 58 aa, artificial sequence
  Modified bacterial sequence
VDAKYAKETIDAWNEIDHLPNLTLDQWLAFINKLDDDPSQSSELLSEAKKLNDSQAPK

SEQ ID NO: 722 - protein, 58 aa, artificial sequence
  Modified bacterial sequence
VDAKYAKEVVAAWTEIDLLPNLTLDQWLAFINKLEDDPSQSSELLSEAKKLNDSQAPK

SEQ ID NO: 723 - protein, 58 aa, artificial sequence
  Modified bacterial sequence
VDAKYAKEVVAAWDEIDALPNLTIEQWLAFINKLSDDPSQSSELLSEAKKLNDSQAPK

SEQ ID NO: 724 - protein, 58 aa, artificial sequence
  Modified bacterial sequence
VDAKYAKETLEAWREIDSLPNLTLEQWLAFINKLDDDPSQSSELLSEAKKLNDSQAPK

SEQ ID NO: 725 - protein, 58 aa, artificial sequence
  Modified bacterial sequence
VDAKYAKEVIKAWNEIDHLPNLTLDQWLAFINKLDDDPSQSSELLSEAKKLNDSQAPK

SEQ ID NO: 726 - protein, 58 aa, artificial sequence
  Modified bacterial sequence
VDAKYAKEVLEAWTEIDKLPNLTIDQWLAFINKLDDDPSQSSELLSEAKKLNDSQAPK

SEQ ID NO: 727 - protein, 58 aa, artificial sequence
  Modified bacterial sequence
VDAKYAKETLEAWDEIDKLPNLTIDQWLAFINKLDDDPSQSSELLSEAKKLNDSQAPK

SEQ ID NO: 728 - protein, 58 aa, artificial sequence
  Modified bacterial sequence
VDAKYAKEVIEAWNEIDKLPNLTIDQWLAFINKLDDDPSQSSELLSEAKKLNDSQAPK

SEQ ID NO: 729 - protein, 58 aa, artificial sequence
  Modified bacterial sequence
VDAKYAKETIDAWNEIDKLPNLTLEQWLAFINKLDDDPSQSSELLSEAKKLNDSQAPK

SEQ ID NO: 730 - protein, 58 aa, artificial sequence
  Modified bacterial sequence
VDAKYAKETLDAWDEIDALPNLTIDQWLAFINKLEDDPSQSSELLSEAKKLNDSQAPK

SEQ ID NO: 731 - protein, 58 aa, artificial sequence
  Modified bacterial sequence
VDAKYAKEVLSAWNEIDHLPNLTIQQWLAFINKLDDDPSQSSELLSEAKKLNDSQAPK

SEQ ID NO: 732 - protein, 58 aa, artificial sequence
  Modified bacterial sequence
VDAKYAKEVIQANDEIDKLPNLTIEQWLAFIHKLHDDPSQSSELLSEAKKLNDSQAPK

SEQ ID NO: 733 - protein, 58 aa, artificial sequence
  Modified bacterial sequence
VDAKYAKEHLDAWDEIDHLPNLTIQQWLAFINKLADDPSQSSELLSEAKKLNDSQAPK

SEQ ID NO: 734 - protein, 58 aa, artificial sequence
  Modified bacterial sequence
VDAKYAKEVIQAWNEIDQLPNLTIEQWLAFINKLDDDPSQSSELLSEAKKLNDSQAPK

SEQ ID NO: 735 - protein, 58 aa, artificial sequence
  Modified bacterial sequence
VDAKYAKEVIEAWNEIDYLPNLTIAQWIAFINKLDDDPSQSSELLSEAKKLNDSQAPK

SEQ ID NO: 736 - protein, 58 aa, artificial sequence
  Modified bacterial sequence
VDAKYAKETIQAWDEIDRLPNLTLQQWLAFINKLDDDPSQSSELLSEAKKLNDSQAPK

SEQ ID NO: 737 - protein, 58 aa, artificial sequence
  Modified bacterial sequence
VDAKYAKETIQAWDEIDKLPNLTIEQWLAFINKLDDDPSQSSELLSEAKKLNDSQAPK

SEQ ID NO: 738 - protein, 58 aa, artificial sequence
  Modified bacterial sequence
VDAKYAKETLDAWAEIDHLPNLTIEQWLAFINKLDDDPSQSSELLSEAKKLNDSQAPK

SEQ ID NO: 739 - protein, 58 aa, artificial sequence
  Modified bacterial sequence
VDAKYAKEVIEAWDEIDKLPNLTLNQWLAFINKLDDDPSQSSELLSEAKKLNDSQAPK

SEQ ID NO: 740 - protein, 58 aa, artificial sequence
  Modified bacterial sequence
VDAKYAKEVLDAWNEIDQLPNLTIEQWLAFINKLDDDPSQSSELLSEAKKLNDSQAPK

SEQ ID NO: 741 - protein, 58 aa, artificial sequence
  Modified bacterial sequence
VDAKYAKEVLHAWNEIDHLPNLTIEQWLAFIEKLEDDPSQSSELLSEAKKLNDSQAPK

SEQ ID NO: 742 - protein, 58 aa, artificial sequence
  Modified bacterial sequence
VDAKYAKEVIEAWQEIDKLPNLTIDQWLAFINKLDDDPSQSSELLSEAKKLNDSQAPK

SEQ ID NO: 743 - protein, 58 aa, artificial sequence
  Modified bacterial sequence
VDAKYAKEVVDAWNEIDQLPNLTIEQWLAFINKLDDDPSQSSELLSEAKKLNDSQAPK

SEQ ID NO: 744 - protein, 58 aa, artificial sequence
  Modified bacterial sequence
VDAKYAKEQIEAWNEIDALPNLTIEQWLAFINKLADDPSQSSELLSEAKKLNDSQAPK

SEQ ID NO: 745 - protein, 60 aa, artificial sequence
  Modified bacterial sequence
VDAKYAKETITAWDEIDKLPNLTIEQWLAFIGKLEDDPSQSSELLAEAKKLNDAQAPKVD

SEQ ID NO: 746 - protein, 60 aa, artificial sequence
  Modified bacterial sequence
AEAKYAKEVIEAWNEIDRLPNLTIEQWLAFINKLDDDPSQSSELLSEAKKLNDSQAPKVD

SEQ ID NO: 747 - protein, 60 aa, artificial sequence
  Modified bacterial sequence
AEAKYAKEVLEAWNEIDRLPNLTIEQWLAFINKLDDDPSQSSELLSEAKKLNDSQAPKVD

SEQ ID NO: 748 - protein, 60 aa, artificial sequence
  Modified bacterial sequence
AEAKYAKEVLEAWDEIDRLPNLTLDQWLAFINKLDDDPSQSSELLSEAKKLNDSQAPKVD

SEQ ID NO: 749 - protein, 60 aa, artificial sequence
  Modified bacterial sequence
AEAKYAKEVLDAWDEIDKLPNLTLEQWLAFINKLDDDPSQSSELLSEAKKLNDSQAPKVD

SEQ ID NO: 750 - protein, 60 aa, artificial sequence
  Modified bacterial sequence
AEAKYAKEVLDAWDEIDALPNLTLEQWLAFINKLDDDPSQSSELLSEAKKLNDSQAPKVD

SEQ ID NO: 751 - protein, 60 aa, artificial sequence
  Modified bacterial sequence
AEAKYAKEVIDAWDEIDRLPNLTLDQWLAFINKLDDDPSQSSELLSEAKKLNDSQAPKVD

SEQ ID NO: 752 - protein, 60 aa, artificial sequence
  Modified bacterial sequence
AEAKYAKETLEAWDEIDRLPNLTIEQWLAFINKLDDDPSQSSELLSEAKKLNDSQAPKVD

SEQ ID NO: 753 - protein, 60 aa, artificial sequence
  Modified bacterial sequence
AEAKYAKEVLEAWDEIDRLPNLTIEQWLAFINKLDDDPSQSSELLSEAKKLNDSQAPKVD

SEQ ID NO: 754 - protein, 60 aa, artificial sequence
  Modified bacterial sequence
AEAKYAKEVIDAWNEIDALPNLTLDQWLAFINKLDDDPSQSSELLSEAKKLNDSQAPKVD

SEQ ID NO: 755 - protein, 60 aa, artificial sequence
  Modified bacterial sequence
AEAKYAKEVLDAWDEIDKLPNLTIDQWLAFINKLDDDPSQSSELLSEAKKLNDSQAPKVD

SEQ ID NO: 756 - protein, 60 aa, artificial sequence
  Modified bacterial sequence
AEAKYAKEVLEAWDEIDHLPNLTLDQWLAFINKLDDDPSQSSELLSEAKKLNDSQAPKVD

SEQ ID NO: 757 - protein, 60 aa, artificial sequence
  Modified bacterial sequence
AEAKYAKEVLEAWDEIDALPNLTIEQWLAFINKLDDDPSQSSELLSEAKKLNDSQAPKVD

SEQ ID NO: 758 - protein, 58 aa, artificial sequence [sequence omitted]

SEQ ID NO: 759 - protein, 46 aa, artificial sequence
  Modified bacterial sequence
LAEAKEAANAELDSYGVSDFYKRLIDKAKTVEGVEALKDAILAALP

SEQ ID NO: 760 - protein, 1676 aa, Homo sapiens
MGLLGILCFLIFLGKTWGQEQTYVISAPKIFRVGASENIVIQVYGYTEAFDATISIKSYPDKKFSYSSGHVHLSSENKFQNSAILTIQPKQLPGGQNPVSYVYLEVVSKHFSKSKRMPITYDNGFLFIHTDKPVYTPDQSVKVRVYSLNDDLKPAKRETVLTFIDPEGSEVDMVEEIDHIGIISFPDFKIPSNPRYGMWTIKAKYKEDFSTTGTAYFEVKEYVLPHFSVSIEPEYNFIGYKNFKNFEITIKARYFYNKVVTEADVYITFGIREDLKDDQKEMMQTAMQNTMLINGIAQVTFDSETAVKELSYYSLEDLNNKYLYIAVTVIESTGGFSEEAEIPGIKYVLSPYKLNLVATPLFLKPGIPYPIKVQVKDSLDQLVGGVPVTLNAQTIDVNQETSDLDPSKSVTRVDDGVASFVLNLPSGVTVLEFNVKTDAPDLPEENQAREGYRAIAYSSLSQSYLYIDWTDNHKALLVGEHLNIIVTPKSPYIDKITHYNYLILSKGKIIHFGTREKFSDASYQSINIPVTQNMVPSSRLLVYYIVTGEQTAELVSDSVWLNIEEKCGNQLQVHLSPDADAYSPGQTVSLNMATGMDSWVALAAVDSAVYGVQRGAKKPLERVFQFLEKSDLGCGAGGGLNNANVFHLAGLTFLTNANADDSQENDEPCKEILRPRRTLQKKIEEIAAKYKHSVVKKCCYDGACVNNDETCEQRAARISLGPRCIKAFTECCVVASQLRANISHKDMQLGRLHMKTLLPVSKPEIRSYFPESWLWEVHLVPRRKQLQFALPDSLTTWEIQGVGISNTGICVADTVKAKVFKDVFLEMNIPYSVVRGEQIQLKGTVYNYRTSGMQFCVKMSAVEGICTSESPVIDHQGTKSSKCVRQKVEGSSSHLVTFTVLPLEIGLHNINFSLETWFGKEILVKTLRVVPEGVKRESYSGVTLDPRGIYGTISRRKEFPYRIPLDLVPKTEIKRILSVKGLLVGEILSAVLSQEGINILTHLPKGSAEAELMSVVPVFYVFHYLETGNHWNIFHSDPLIEKQKLKKKLKEGMLSIMSYRNADYSYSVWKGGSASTWLTAFALRVLGQVNKYVEQNQNSICNSLLWLVENYQLDNGSFKENSQYQPIKLQGTLPVEARENSLYLTAFTVIGIRKAFDICPLVKIDTALIKADNFLLENTLPAQSTFTLAISAYALSLGDKTHPQFRSIVSALKREALVKGNPPIYRFWKDNLQHKDSSVPNTGTARMVETTAYALLTSLNLKDINYVNPVIKWLSEEQRYGGGFYSTQDTINAIEGLTEYSLLVKQLRLSMDIDVSYKHKGALHNYKMTDKNFLGRPVEVLLNDDLIVSTGFGSGLATVHVTTVVHKTSTSEEVCSFYLKIDTQDIEASHYRGYGNSDYKRIVACASYKPSREESSSGSSHAVMDISLPTGISANEEDLKALVEGVDQLFTDYQIKDGHVILQLNSIPSSDFLCVRFRIFELFEVGFLSPATFTVYEYHRPDKQCTMFYSTSNIKIQKVCEGAACKCVEADCGQMQEELDLTISAETRKQTACKPEIAYAYKVSITSITVENVFVKYKATLLDIYKTGEAVAEKDSEITFIKKVTCTNAELVKGRQYLIMGKEALQIKYNFSFRYIYPLDSLTWIEYWPRDTTCSSCQAFLANLDEFAEDIFLNGC

SEQ ID NO: 761 - protein, 170 aa, Ornithodoros moubata
MDSESDCTGSEPVDAFQAFSEGKEAYVLVRSTDPKARDCLKGEPAGEKQDNTLPVMMTFKNGTDWASTDWTFTLDGAKVTATLGNLTQNREVVYDSQSHHCHVDKVEKEVPDYEMWMLDAGGLEVEVECCRQKLEELASGRNQMYPHLKDCGGGGSENLYFQGSHHHHHH

SEQ ID NO: 762 - protein, 1676 aa, Macaca fascicularis
  misc_feature (63)..(63): Xaa can be any naturally occurring amino acid
  misc_feature (1346)..(1346): Xaa can be any naturally occurring amino acid
MGLLGILCFLIFLGKTWGQEQTYVISAPKIFRVGASENIVIQVYGYTEAFDATISIKSYPDKXFSYSSGHVHLSSENKFQNSAVLTIQPKQLPGGQNQVSYVYLEVVSKHFSKSKKIPITYDNGFLFIHTDKPVYTPDQSVKVRVYSLNDDLKPAKRETVLTFIDPEGSEIDMVEEIDHIGIISFPDFKIPSNPRYGMWTIQAKYKEDFSTTGTAFFEVKEYVLPHFSVSVEPESNFIGYKNFKNFEITIKARIFYNKVVTEADVYITFGIREDLKDDQKEMMQTAMQNTMLINGIAEVTFDSETAVKELSYYSLEDLNNKYLYIAVTVIESTGGFSEEAEIPGIKYVLSPYKLNLVATPLFLKPGIPYSIKVQVKDALDQLVGGVPVTLNAQTIDVNQETSDLEPRKSVTRVDDGVASFVVNLPSGVTVLEFNVKTDAPDLPDENQAREGYRAIAYSSLSQSYLYIDWTDNHKALLVGEYLNIIVTPKSPYIDKITHYNYLILSKGKIIHFGTREKLSDASYQSINIPVTQNMVPSSRLLVYYIVTGEQTAELVSDSVWLNIEEKCGNQLQVHLSPDADTYSPGQTVSLNMVTGMDSWVALTAVDSAVYGVQRRAKKPLERVFQFLEKSDLGCGAGGGLNNANVFHLAGLTFLTNANADDSQENDEPCKEIIRPRRMLQEKIEEIAAKYKHLVVKKCCYDGVRINHDETCEQRAARISVGPRCVKAFTECCVVASQLRANNSHKDLQLGRLHMKTLLPVSKPEIRSYFPESWLWEVHLVPRRKQLQFALPDSVTTWEIQGVGISNSGICVADTIKAKVFKDVFLEMNIPYSVVRGEQVQLKGTVYNYRTSGMQFCVKMSAVEGICTSESPVIDHQGTKSSKCVRQKVEGSSNHLVTFTVLPLEIGLQNINFSLETSFGKEILVKSLRVVPEGVKRESYSGITLDPRGIYGTISRRKEFPYRIPLDLVPKTEIKRILSVKGLLVGEILSAVLSREGINILTHLPKGSAEAELMSVVPVFYVFHYLETGNHWNIFHSDPLIEKRNLEKKLKEGMVSIMSYRNADYSYSVWKGGSASTWLTAFALRVLGQVHKYVEQNQNSICNSLLWLVENYQLDNGSFKENSQYQPIKLQGTLPVEARENSLYLTAFTVIGIRKAFDICPLVKINTALIKADTFLLENTLPAQSTFTLAISAYALSLGDKTHPQFRSIVSALKREALVKGNPPIYRFWKDSLQHKDSSVPNTGTARMVETTAYALLTSLNLKDINYVNPIIKWLSEEQRYGGGFYSTQDTINAIEGLTEYSLLVKQLRLNMDIDVAYKHKGPLHNYKMTDKNFLGRPVEVLLNDDXVVSTGFGSGLATVHVTTVVHKTSTSEEVCSFYLKIDTQDVEASHYRGYGNSDYKRIVACASYKPSKEESSSGSSHAVMDISLPTGINANEEDLKALVEGVDQLFTDYQIKDGHVILQLNSIPSSDFLCVRFRIFELFEVGFLSPATFTVYEYHRPDKQCTMFYSTSNIKIQKVCEGATCKCIEADCGQMQKELDLTISAETRKQTACNPEIAYAYKVIITSITTENVFVKYKATLLDIYKTGEAVAEKDSEITFIKKVTCTNAELVKGRQYLIMGKEALQIKYNFTFRYIYPLDSLTWIEYWPRDTTCSSCQAFLANLDEFAEDIFLNGC